European Patent Application EP 4 136 964 A1, published February 22, 2023. Title: A plant belonging to genus Nicotiana with low alkaloid content and method of producing the same. Applicant: JAPAN TOBACCO INC. The sequence listing filed with the application follows.

SEQUENCE LISTING (70 sequences)

SEQ ID NO: 1 - DNA, 1947 bp, Nicotiana sylvestris
atggcaactggtatcgcttcaggatgcggacagttacatttgaggaagcctgtctacttgaggaatagctatggaaataaagctcactctcattccaatgtgattctcaacggcacgcaaaaccagatcgcttggtctagttgggtttcaaatgtcttgcgagttaatagaagtagctatccacaatgtcaagtgataaaaacaaactggaagtctcggcgaggaacaatcaaatctagccagcagagagatgggtcagttactaggtacttcgatttcattgtgattggtagtggaattgctggccttcgatatgcacttgaggttgccaagcatggaactgtggctgtgataaccaaggctgagccacatgagagtagcactaactatgctcaaggtggtgtaagtgctgtgctctgccctttggattcagtggagaaccacatacaagatacaattgtggcaggtgcttacctctgtgataaggagactgttaaagtagtgtgtactgaaggacctgagagaattagagaactgatcgctataggtgcttcattcgatcatggggaggacggaaatctggatctagccagggaaggaggccactcccatcgtcgaattgtccatgctgctgatatgactggcagagagattgaaagagccttattagaggcagtgtttaagaatcctaatatacatgtgtttcaacaccattttgctatcgatttgttgaccactcaggatggttctgacgtagtatgtcatggcgttgatactatacacacggaaacgaaggaggttataagattcatttcaaaagtgactttgctagcatcaggtggagttggacatatctatccaagtactactaatccgacggttgcaactggtgatggaatggctatggctcatcgagctcaagctgtaatttccaacatggagtttgtgcaattccacccaactgccttggctgatgaagggcttcccaacataccaagtgccagagagaatgcttttttgataactgaagctgtcagaggtgatggaggcatcctttataacttagatatggaaagatttatgccaatgtatgatgaaagagcagaacttgccccgagagatgtggtagcaagaagtatagatgaccagctcaaaaagcgtggcgaaaagtatgttcttcttgatatcagtcacaagcccagagagaaggttctgtcccattttcctaatatagctgctgagtgtctccgccatgggttagacataacacagcagccgattccggtggttcctgctgctcactacatgtgtggtggagtccgtgctggactcgagggtgagactaatgtgcaaggtctttatgtggcaggtgaagttgcatgtactggtttacatggtgcaaaccgacttgctagcaactcattgcttgaagcactagtgtttgcacgaagagctgtacagccttcaattgatcatgtgaacgtgtctagaattgataacggtgcatcaagttggtggccgcggcctgtagcccccatggcactaggagatacagtacttaacaaagtcatccgtcggacaagggaagtgaggaaagaactacagtcaatcatgtgggaatatgttggaattgttaggtctacctcaagactaaatactgctgagaagagaatcaaagagttggagttggaatgggaaacatacctgtttcagcatggctgggaaccaacaatggttggagtagaggcttgtgagatgaggaatctcttctgttgtgccaacctggtagttagcagtgctctttctcgacaagagagtcgtgggcttcactacaccactgattttcctcatgttgaggaaagcgagaggttgccaacggttatctttccttctcagcgaaatagcacatggagcacacggcaattacacgcgcagccgataagttag

SEQ ID NO: 2 - protein, 648 aa, Nicotiana sylvestris
MATGIASGCGQLHLRKPVYLRNSYGNKAHSHSNVILNGTQNQIAWSSWVSNVLRVNRSSYPQCQVIKTNWKSRRGTIKSSQQRDGSVTRYFDFIVIGSGIAGLRYALEVAKHGTVAVITKAEPHESSTNYAQGGVSAVLCPLDSVENHIQDTIVAGAYLCDKETVKVVCTEGPERIRELIAIGASFDHGEDGNLDLAREGGHSHRRIVHAADMTGREIERALLEAVFKNPNIHVFQHHFAIDLLTTQDGSDVVCHGVDTIHTETKEVIRFISKVTLLASGGVGHIYPSTTNPTVATGDGMAMAHRAQAVISNMEFVQFHPTALADEGLPNIPSARENAFLITEAVRGDGGILYNLDMERFMPMYDERAELAPRDVVARSIDDQLKKRGEKYVLLDISHKPREKVLSHFPNIAAECLRHGLDITQQPIPVVPAAHYMCGGVRAGLEGETNVQGLYVAGEVACTGLHGANRLASNSLLEALVFARRAVQPSIDHVNVSRIDNGASSWWPRPVAPMALGDTVLNKVIRRTREVRKELQSIMWEYVGIVRSTSRLNTAEKRIKELELEWETYLFQHGWEPTMVGVEACEMRNLFCCANLVVSSALSRQESRGLHYTTDFPHVEESERLPTVIFPSQRNSTWSTRQLHAQPIS

SEQ ID NO: 3 - DNA, 1947 bp, Nicotiana tabacum
atggcaactggtatcgcttcaggatgcggacagttacatttgaggaagcctgtctacttgaggaatagctatggaaataaagctcactctcattccaatgtgattctcaacggcacgcaaaaccagatcgcttggtctagttgggtttcaaatgtcttgcgagttaatagaagtagctatccacaatgtcaagtgataaaaacaaactggaagtctcggcgaggaacaatcaaatctagccagcagagagatggatcagttactaggtacttcgatttcattgtgattggtagtggaattgctggccttcgatatgcacttgaggttgccaagcatggaactgtggctgtgataaccaaggctgagccacatgagagtagcactaactatgctcaaggtggtgtaagtgctgtgctctgccctttggattcagtggagaaccacatacaagatacaattgtggcaggtgcttacctctgtgataaggagactgttaaagtagtgtgtactgaaggacctgagagaattagagaactgatcgctataggtgcttcattcgatcatggggaggacggaaatctggatctagccagggaaggaggccactcccatcgtcgaattgtccatgctgctgatatgactggcagagagattgaaagagccttattagaggcagtgtttaagaatcctaatatacatgtgtttcaacaccattttgctatcgatttgttgaccactcaggatggttctgacgtagtatgtcatggcgttgatactatacacacggaaacgaaggaggttataagattcatttcaaaagtgactttgctagcatcaggtggagttggacatatctatccaagtactactaatccgacggttgcaactggtgatggaatggctatggctcatcgagctcaagctgtaatttccaacatggagtttgtgcaattccacccaactgccttggctgatgaagggcttcccaacataccaagtgccagagagaatgcttttttgataactgaagctgtcagaggtgatggaggcatcctttataacttagatatggaaagatttatgccaatgtatgatgaaagagcagaacttgccccgagagatgtggtagcaagaagtatagatgaccagctcaaaaagcgtggcgaaaagtatgttcttcttgatatcagtcacaagcccagagagaaggttctgtcccattttcctaatatagctgctgagtgtctccgccatgggttagacataacacagcagccgattccggtggttcctgctgctcactacatgtgtggtggagtccgtgctggactcgagggtgagactaatgtgcaaggtctttatgtggcaggtgaagttgcatgtactggtttacatggtgcaaaccgacttgctagcaactcattgcttgaagcactagtgtttgcacgaagagctgtacagccttcaattgatcatgtgaacgtgtctagaattgataacggtgcatcaagttggtggccgcggcctgtagcccccctggcactaggagatacagtacttaacaaagtcatccgtcggacaagggaagtgaggaaagaactacagtcaatcatgtgggaatatgttggaattgttaggtctacctcaagactaaatactgctgagaagagaatcaaagagttggagttggaatgggaaacatacctgtttcagcatggctgggaaccaacaatggttggagtagaggcttgtgagatgaggaatctcttctgttgtgccaacctggtagttagcagtgctctttctcgacaagagagtcgtgggcttcactacaccactgattttcctcatgttgaggaaagcgagaggttgccaacggttatctttccttctcagcgaaatagcacatggagcacacggcaattacacgcgcagccgataagttag

SEQ ID NO: 4 - DNA, 1947 bp, Nicotiana tabacum
atggcaactggtatcgcttcaggatgcggacagttacacttgaggaagcctgtctacttgaggaatagctatggaaataaagctcactgtcattccaatgtgattctcaacggcacgcaaaaccagatcgcttggtctagttgggtttcaaatgtcttgcgagttaatagaagtagctatccagaatgtcaagtgatcaagacaaactggaagtctagccgaggaacaatcaaatcgtgccagcagagagatggatcagttactaggtacttcgatttcactgtgattggtagtggaattgctggccttcgatatgcacttgaggttgccaagcatggaactgtggctgtaataaccaaggctgagccacatgagagtagcactaactatgctcaaggtggtgtaagtgctgtgctctgccctttggattcagtggagagccatatgcaagatacaattgtggcaggtgcttatctctgtgataaggagactgttagagtagtgtgtactgaaggacctgagagaattagagaactgatcgctatgggtgcttcattcgatcatggggaggacggaaatctggatctagccagggaaggaggccactcccatcgtcgaattgtccatgctgctgatatgactggcagagagatagaaagagctctattagaggcagtttttaagaatcctaatatacatgtgtttcaacaccattttgctatagatttgttgaccactcaggatggttctgacatagtatgtcatggcgttgatactatacacacggaaacgaaggaggttataagattcatttcaaaagtgactttgctggcatcaggtggagttggacatatctatccaagtactactaatccgacggttgcaactggtgatggaatggctatggctcatcgagctcaagctgtaatttccaacatggagtttgtgcaattccacccaactgccttggctgatgaaggccttcccaacataccaagtgccagagagaatgcttttttgataactgaagctgtcagaggtgatggaggcatcctttacaacttagatatggaaagatttatgccaatgtatgatgaaagagcagaacttgccccgagagatgtggtagcaagaagtatagatgaccagctcaaaaagcgtggcgaaaagtatgttcttcttgatatcagtcacaagcccagagagaaggttctttctcattttcctaatatagctgctgagtgtctccgccatgggttagacataacacagcagccgattccggtggttcctgctgctcactacatgtgtggtggagtccgtgctggactcgagggtgagactaatgtgcaaggtctttatgtggcaggtgaagttgcatgtactggtttacatggtgctaaccgacttgctagcaactcattgcttgaagcactagtgtttgcacgaagagctgtacagccttcaattgatcatgtgaacgtgtctagaattgatcacggtgcttcaagttggtggccgcggcctgtagcccccatggtactaggagatacagtacttaacaaagtcatctgtcggacaagggaagtgaggaaagaactacagtcaatcatgtgggaatatgttggaattgttaggtctaactcaagactaaacactgctgagaagagaatcagagagttggagttggaatgggaaacatacctatttcagcatggctgggaaccaacaatggttggagtagaggcttgtgagatgaggaatctcttctgttgtgccaacttggtagttagcagtgctctttctcgacatgagagtcgtgggcttcactacaccactgattttcctcatgttgaggaaagcgagaggttgccaacggtcatttttccttctcagcgaaataactcatggagctcacgccaattacacgcgcagccgataagttag

SEQ ID NO: 5 - protein, 648 aa, Nicotiana tabacum
MATGIASGCGQLHLRKPVYLRNSYGNKAHSHSNVILNGTQNQIAWSSWVSNVLRVNRSSYPQCQVIKTNWKSRRGTIKSSQQRDGSVTRYFDFIVIGSGIAGLRYALEVAKHGTVAVITKAEPHESSTNYAQGGVSAVLCPLDSVENHIQDTIVAGAYLCDKETVKVVCTEGPERIRELIAIGASFDHGEDGNLDLAREGGHSHRRIVHAADMTGREIERALLEAVFKNPNIHVFQHHFAIDLLTTQDGSDVVCHGVDTIHTETKEVIRFISKVTLLASGGVGHIYPSTTNPTVATGDGMAMAHRAQAVISNMEFVQFHPTALADEGLPNIPSARENAFLITEAVRGDGGILYNLDMERFMPMYDERAELAPRDVVARSIDDQLKKRGEKYVLLDISHKPREKVLSHFPNIAAECLRHGLDITQQPIPVVPAAHYMCGGVRAGLEGETNVQGLYVAGEVACTGLHGANRLASNSLLEALVFARRAVQPSIDHVNVSRIDNGASSWWPRPVAPLALGDTVLNKVIRRTREVRKELQSIMWEYVGIVRSTSRLNTAEKRIKELELEWETYLFQHGWEPTMVGVEACEMRNLFCCANLVVSSALSRQESRGLHYTTDFPHVEESERLPTVIFPSQRNSTWSTRQLHAQPIS

SEQ ID NO: 6 - protein, 648 aa, Nicotiana tabacum
MATGIASGCGQLHLRKPVYLRNSYGNKAHCHSNVILNGTQNQIAWSSWVSNVLRVNRSSYPECQVIKTNWKSSRGTIKSCQQRDGSVTRYFDFTVIGSGIAGLRYALEVAKHGTVAVITKAEPHESSTNYAQGGVSAVLCPLDSVESHMQDTIVAGAYLCDKETVRVVCTEGPERIRELIAMGASFDHGEDGNLDLAREGGHSHRRIVHAADMTGREIERALLEAVFKNPNIHVFQHHFAIDLLTTQDGSDIVCHGVDTIHTETKEVIRFISKVTLLASGGVGHIYPSTTNPTVATGDGMAMAHRAQAVISNMEFVQFHPTALADEGLPNIPSARENAFLITEAVRGDGGILYNLDMERFMPMYDERAELAPRDVVARSIDDQLKKRGEKYVLLDISHKPREKVLSHFPNIAAECLRHGLDITQQPIPVVPAAHYMCGGVRAGLEGETNVQGLYVAGEVACTGLHGANRLASNSLLEALVFARRAVQPSIDHVNVSRIDHGASSWWPRPVAPMVLGDTVLNKVICRTREVRKELQSIMWEYVGIVRSNSRLNTAEKRIRELELEWETYLFQHGWEPTMVGVEACEMRNLFCCANLVVSSALSRHESRGLHYTTDFPHVEESERLPTVIFPSQRNNSWSSRQLHAQPIS

SEQ ID NO: 7 - DNA, 21 bp, Artificial Sequence
  Synthetic Primer
tgcacgaccataatacttcac

SEQ ID NO: 8 - DNA, 21 bp, Artificial Sequence
  Synthetic Primer
aagctcgtgacctgtgatatg

SEQ ID NO: 9 - DNA, 21 bp, Artificial Sequence
  Synthetic Primer
catgacgtgacacaattctag

SEQ ID NO: 10 - DNA, 21 bp, Artificial Sequence
  Synthetic Primer
gtgatatgtttgactgggcac

SEQ ID NO: 11 - DNA, 15 bp, Artificial Sequence
  Synthetic Primer
ctaggtacttcgatt

SEQ ID NO: 12 - DNA, 22 bp, Artificial Sequence
  Synthetic Primer
gtatgtggttctccactgaatc

SEQ ID NO: 13 - DNA, 21 bp, Artificial Sequence
  Synthetic Primer
atgtgtttcaacaccattttg

SEQ ID NO: 14 - DNA, 20 bp, Artificial Sequence
  Synthetic Primer
acaacatcaaatccttgctg

SEQ ID NO: 15 - DNA, 22 bp, Artificial Sequence
  Synthetic Primer
ccaacatccattacatacttag

SEQ ID NO: 16 - DNA, 21 bp, Artificial Sequence
  Synthetic Primer
caccagttgcaacctataatc

SEQ ID NO: 17 - DNA, 22 bp, Artificial Sequence
  Synthetic Primer
gaaagatttatgccaatgtatg

SEQ ID NO: 18 - DNA, 21 bp, Artificial Sequence
  Synthetic Primer
tctgggcttgtgactgatatc

SEQ ID NO: 19 - DNA, 22 bp, Artificial Sequence
  Synthetic Primer
ctagaattgataacggtgcatc

SEQ ID NO: 20 - DNA, 23 bp, Artificial Sequence
  Synthetic Primer
gaggtagacctaacaattccaac

SEQ ID NO: 21 - DNA, 28 bp, Artificial Sequence
  Synthetic Primer
cacctgaggaatagctatggaaataaag

SEQ ID NO: 22 - DNA, 24 bp, Artificial Sequence
  Synthetic Primer
tgaaatcgaagtacctagtaactg

SEQ ID NO: 23 - DNA, 26 bp, Artificial Sequence
  Synthetic Primer
caccagagagtcgtgggcttcactac

SEQ ID NO: 24 - DNA, 21 bp, Artificial Sequence
  Synthetic Primer
ctaacttatcggctgcgcgtg

SEQ ID NO: 25 - DNA, 30 bp, Artificial Sequence
  Synthetic Primer
taagagacaggcgaggaacaatcaaatcta

SEQ ID NO: 26 - DNA, 30 bp, Artificial Sequence
  Synthetic Primer
taagagacaggggaaatagtctccaaatta

SEQ ID NO: 27 - DNA, 30 bp, Artificial Sequence
  Synthetic Primer
taagagacaggcagagagattgaaagagcc

SEQ ID NO: 28 - DNA, 30 bp, Artificial Sequence
  Synthetic Primer
taagagacagctgaatagttcaattgcgac

SEQ ID NO: 29 - DNA, 29 bp, Artificial Sequence
  Synthetic Primer
taagagacagaggatgcggacagttacac

SEQ ID NO: 30 - DNA, 30 bp, Artificial Sequence
  Synthetic Primer
taagagacaggccatggataatagtttgac

SEQ ID NO: 31 - DNA, 30 bp, Artificial Sequence
  Synthetic Primer
taagagacagtaaacatcgcgctaataatc

SEQ ID NO: 32 - DNA, 30 bp, Artificial Sequence
  Synthetic Primer
taagagacagtagacttccagtttgtcttg

SEQ ID NO: 33 - DNA, 30 bp, Artificial Sequence
  Synthetic Primer
taagagacagcagagagatagaaagagctc

SEQ ID NO: 34 - DNA, 29 bp, Artificial Sequence
  Synthetic Primer
taagagacagcaagtaagagcgcagaagc

SEQ ID NO: 35 - DNA, 9075 bp, Nicotiana sylvestris
attttggtgcacctgaaaatgatataccggattactaaacttatattttatgtttttttaatgtaatttcaattttagtgtatcctcctttgatgtacttttaattttaatgtatttttattttatgtattgttaattttctttttaaattttagttttcacttttcaattttagcaacattagatatcttacatttgcatttttcatttttaaataattgttatatttctttttatacaattataataataataaaattaacttataattttatatataatatatataaaaattaatatatcaaaaaaataggatataaaattaaaattataaagatcttaatataaaaattaactatatacacaatatatgataaattaaagtccaaaaaaataaaaataaaaaagaataaaataataataaatcaaatttggtgttgatgaatagtgtcacaccaaatttggtgtgagactattcacatactaaaatggtgcaaaatttgatgttccattggagcaaaaaaaatactaaatcttacaccaaatttagatttgctgcaaaaaatagtgcaccattggagatgccctaagaccatctccaaggctgcattatagagcatgaatagtgttgcaccaaatttggtgcaacactattcatcactccatatttggtttattattattttattcaatctttttattttttggacttttaatttatcatatattgtgtatataattaatttttatattaagatctttataattttaattttatatcctattttttgatatattaattttgtatatattatatttatataaaattataagttaattttattattattataattgtataaaaagagatataaccgttatttaaaaataaaaaatgcaaatgtaagatatctaatgatgcgcatttcgcacttcgtaatgcattaatcgagcatttatgggagaataaaggcgtaagttaaatatttatgtggtacttaaattaaatttgactatgatgtaatatttatttaattatcttttatcaatgatttcacttttagttgatttatcctttaaaaaaattttgtaataaatgattatataagtggtgaatgtgaattatatataatgaatatggaaaaaagaaaaaagatagtattagtttgaaggaaataaaaaatgaaaagtaaatagaagataataatataatatagaagagagagaagatttggtgtaaaaaattgtgtaatggttgaattaaatatggtgttacatcattttgatgtgaaatttggtgttagggttgcagatggcctaagaggagtgacctattgtctagatagtaataatgtagttttgtttaactaaagtagtggttatatgttcaactttagaggtttttgcttttacttgtatatatttttttcctggtgaataaacttttagttacccaaaaataataataattgagttaaaagaattgttacaaagaaacacaaataaggtaatattgtaaaccacgaagaaggtcagtgtgtgagatacaaaatgtcaggagaggtgtctgaaattattgtttttggcattgctgagaacattaacaataagaaaaaagcattaacaatcaacatatattcaaattggtaaaaaaacatgttcaaattggtgggttagaataagttaggacccattaactatttaatcagtttaaatttaggtagactctattatttgattgtagatataaaagataatattaaagagagaaactaccaacccctgtaacattaaaaaaaagttagaaacaatgttcattagaagatccaaaaggcaaaagataaaaataaagagaaataagatgaccgaaaccaacaattgatcgagcaaacaataaacaaagaggatagagaagaaaaactcacgaggaatcgagaaagacaaaggagaaggaaagagatatggaaaaatgaaaatcttagtttcagatggagtgctgaaggcaaaagggttaggaaaaattaaatcacgtgggaattggaagtgaataaatgtaaggccatagcacctcaaaatatacacgcagtcagaggctggacgggaccaggatttcaagtttatgggttcggaattccaatagtttgaagttactgtgttctagattaataatttatacatattcaatgacatttttaagacaaatatagtgttcgaaccaaagctactaggttcggccgaacccgctcccgccactctagctccacgcatgcagcaattaagtactccataatgattgaattacacataaacaaatgcataagcaacgtggtgtttgcaagtgaacagctgaaagtccatagcacctcaaaaaagactaaggtaagggtatcaatacaagcagcaattaagtaataaggaccaaatcacacagtatccctaaacaaatacttattaagtgatgaggtacgaatcggaatcgcacagtatcactaaacaaatgcatacaccacgtgggtgttatggaagtgaagtcataagcacctcaaaaatggaccaaattacacagttatccctaaacaaatgcataataccgaaactacccatgcacgaccataatacttcacttattatatagttatggcttctgcttccttggccaacaatcagttcatctctaacttcgaattccagttccattttcacttgacacacttcgaagcgccatctttgctactttaaggtaattgtatatttcaaaagtttgttttgcttatctgttttggaatgacagcggtaattgtgttgtttaacaaatttacatgctccaaatgaatggaagaagagttctaacttcaagaccatggccagaggccagttgttaattcctaagatcatcctgaacaaaatcttctctatatgtagcctctacgtactatattcgttcatgctttaatgtgtaatgcataacaagattttaccttaaatatccagatcgatcatatggcaactggtatcgcttcaggatgcggacagttacatttgaggaagcctgtctacttgaggaatagctatggaaataaagctcactctcattccaatgtgattctcaacggcacgcaaaaccagatcgcttggtacgttttaggggtaaaccagtaatatattttttcatgacgtgacacaattctagaagtagtcatttcctgattccttaggaaaagggaaggttatttcgtcccaatttatatatcatagttacacattcttatatttagtagtaacaatttaactttaaaatacctcttttacccttaatgaaatgatttatagccaaacacatatccattgctcagtttacaccataaatttcaaaaatattcttaaatattgtgcccagtcaaacatatcacataaattgagacattgagacatagaggagtactatgctaattttctgatggtgatatgctttaccaggtctagttgggtttcaaatgtcttgcgagttaatagaagtagctatccacaatgtcaagtgataaaaacaaactggaagtctcggcgaggaacaatcaaatctagccagcagagagatgggtcagttactaggtacttcgatttcattgtgattggtagtggaattgctggccttcgatatgcacttgaggttgccaagcatggaactgtggctgtgataaccaaggctgagccacatgagagtagcactaactatgctcaaggtggtgtaagtgctgtgctctgccctttggattcagtggagaaccacatacaagatacaattgtggcaggtgcttacctctgtgataaggagactgttaaagtaagttcacacgaatatattcagtttaatttggagactatttccccccttttgcttttgctataagtgtatctctcctttaatttctccaggtagtgtgtactgaaggacctgagagaattagagaactgatcgctataggtgcttcattcgatcatggggaggacggaaatctggatctagccagggaaggaggccactcccatcgtcgaattgtccatgctgctgatatgactggcagagagattgaaagagccttattagaggcagtgtttaagaatcctaatatacatgtgtttcaacaccattttgctatcgatttgttgaccactcaggttagtttattagtgtgctatagttgagtaaaggtcgcaattgaactattcagcaaggatttgatgttgtaatttgtatggcaaatgcaggatggttctgacgtagtatgtcatggcgttgatactatacacacggaaacgaaggaggtaagtaacagttgctttcactcatgttgacttttcaacattcttcaaaatgacataaattgattttcttacttgtgtattttaggttataagattcatttcaaaagtgactttgctagcatcaggtggagttggacatatctatccaagtactactaatccgacggtatggtttcaatatcttttcctccaaaatcttgttagttatgattaatgtcatgctccaaaaataaaagatctggacatggcactcgatcgatgctttgaaacttgtgacagagcgaaccaacatccattacatacttagtgcaattagaaatatgagctcgctgccctaaatgcctaaaaaaggattctgtttttatactttgaccatttgtgccaacagaaaagtttaaccctgttgaatgtgggcttgtttaactttctaattcatattgacattatgattataggttgcaactggtgatggaatggctatggctcatcgagctcaagctgtaatttccaacatggagtaagtaatcctcagtagcattatttttattgtacaatatctctgcctctgctttagtgagttttgtgctgtaaaatctgctgacctagatttcatccttttttttttctttcctgatttctgcatcttgttcagcatttcgttcagaatttgcactttcgactaaaaacacaagggtgtgttcaaaaatttgcattattaataacaattctcttcctcgtgttgccaggtttgtgcaattccacccaactgccttggctgatgaagggcttcccaacataccaagtgccagagagaatgcttttttgataactgaagctgtcagaggtgatggaggcatcctttataacttagatatggaaagatttatgccaatgtatgatgaaagagcagaacttgccccgagagatgtggtagcaagaagtatagatgaccagctcaaaaagcgtggcgaaaagtatgttcttcttgatatcagtcacaagcccagagagaaggttctgtcccattttcctaatatagctgctgagtgtctccgccatgggttagacataacacagcagccgattccggtggttcctgctgctcactacatgtgtggtggagtccgtgctggactcgagggtgagactaatgtgcaaggtctttatgtggcaggtgaagttgcatgtactggtttacatggtgcaaaccgacttgctagcaactcattgcttgaagcactagtgtttgcacgaagagctgtacagccttcaattgatcatgtgaacgtgtctagaattgataacggtgcatcaagttggtggccgcggcctgtagcccccatggcactaggagatacagtacttaacaaagtcatccgtcggacaagggaagtgaggaaagaactacagtcaatcatgtgggaatatgttggaattgttaggtctacctcaagactaaatactgctgagaagagaatcaaagagttggagttggaatgggaaacatacctgtttcagcatggctgggaaccaacaatggttggagtagaggcttgtgagatgaggaatctcttctgttgtgccaacctggtagttagcagtgctctttctcgacaagagagtcgtgggcttcactacaccactgattttcctcatgttgaggaaagcgagaggttgccaacggttatctttccttctcagcgaaatagcacatggagcacacggcaattacacgcgcagccgataagttagatatctcttacctatttgccattcttcctgccaaaacatctccagtgcaggacatgatttgtcgattttaccgggttgcaggggtgtatctatcggaaggggtatgggttcatatgaacacatactcctctccatagactatgtataataatgtatatttcttcaatgttatttaaatatgcaagtgtgtcagccaagctcaaagagttcaataattattgggtacatctttacaagtgaaattgtgattttaaatcccatgtctattttgtcgtttttccctttatcttttccgccgaaagtcaaatctcacatttctcttgttggttttcctttcttttcctataaatgggtctacccatgataaaagaaatttcatatttttgttttagtaatttctgaatgcaggttttgacaatttattaaaaacatatcacaggtcacgagctttaattagttaagtaagcaacttgttaaatgtgccagacctgattcttagtgcaattcacccttcttcattttctaggatagttctcctagccagtctgtaacttgctctgttcatggcaaattacaagtgcgtgatagtttggagaccataggaaccctgaactcgaaattggggaaattagagaaaaggcatcgaaaattaaccataaatcagaacaaaatacctcaaaccatgagtacctccatgaattttgctctaaatcatgtaggttttgatcaaatttagctacaaacttgcgttctttggagagagagaattggaaagttaagtccattctagaagaaaatgacgaacatggtccctaatctattgggatttgatcattttggtccttaatgtatgcacttgacctatatagtccttaacctattttaaaaggtgactcttttggtttgaaacactataactaacggtatagttactagcacccactgggcatatggcttataagcatcaatagacgtagccttggaaaggaatggaaattttagggccttgtgagggtagagtaatccttggtaatggacatatttttcttttttataattaaatgatattactgaatggtattccaaacatgtcaattgttcctttttataaggcacataggtggggtaatccggaattgtatagtcgggtataacttctcgagtgatgagatgtttcagagtttaagtaattgaattctcatatatgggataagtattcactttagtgtaaatcttacttccagttaagacaggatattaagcgaccgaagaatacggccaaaagcgggggaagctagaagcgaaaaaatatctcgcttgagtcctccaaaggaagataagagatagtaatgttagtaagaaatagatagaaggataagtatgagaaatgtttaacaattataagctgaagtatggtattatgacaaggttcgtaatcaagaaaaagtgaaggcaagttttaattataaagaggtatgagtcgtaatcacgagaagtgaattttcgacttcaataagagttatcaaaagaccaatctagcccctggattaagaaataccaatattaggtagtaacctaagataacgagatgcaagttagaaactcaaaggatttctgtaatagttggcattgcgacatttacaaagtgaatgatcaggcagtaaaagggtgaatgactatggaacaacctttgagggttagtagaaagagctctccctgagagaagcgtcataagcaaagttaagctcatcaaggtcgagcataccagttatgagtatacaatactacatacatataagttatccaattgctttagtagggaagattaccccaaggcaagttataagccactgaaattgcaaagaattgcaaaaggtggagagttaacgatgtgacctctacaagagtggaattcaagagcataaggagttaattattctcccgagggaagatcgtatgataaagtatcgaggcaaaattatgaggttcgcttagtaacggagcggtaagaaggattacgacaagaggtttgaaaggaataagattgtacttacttagaccctacaaatgtgtaacgactctaatgcataagtacaaacggtagagaaaatgcagtaatgacttcctgactagaggtaccaattgatggtaaataaaactaggcagttgatactcaggaagctagtgtgaggggtaaattaaggcaaaaacatagcctcaagaggagttacttagattttacctatgaagataattgattgagcaatcagtgattagcttatgaagggtctagttatgggttagacgacaaaactcagacgagtcattagatcatgcaaaattacatgttggatcaaaacgtacaaagtttcagcctcgcaagtgcatgatcgcgactctcagaaagtatttcaagacataagcaatggtaggtgaaattccatattatcttttagaaaatcggaaggagcccattgagcttaaaatatgagggaggtgttcaaaagttgtgatcagaagtaatattatagtaaaggagaggtgaaaaacaattagatattattttagatagttcaaaatcacctaaagttctagggagtatatgatgtaatgagctcgcagtcagatatgaacaagagaatcttttctaagtgtgtatacgactaaaatcggagagtccgattttatgatcgttatgacattccacggctcagcttcagaaggcctgaggcacagttcgaagttcgaccccgagggttctcaatgcccaacctcggggtaacgtaaatcgacgactatcttgcataagcgaaaagttcccaaggcgcgtgctcaaagctgacaacacctgcaaatatagtataagttcgtactgtggcattaaatagctgtaccaggttcatatctttgtaataaatgcatatgtactatgttggggttctccctcctatataaaggggacccttgttatttttttcatacatgatatttaatacaaga

SEQ ID NO: 36 - DNA, 9077 bp, Nicotiana tabacum
tggtgcacctgaaaatgatataccggattactaaacttatattttatgtttttttaatgtaatttcaattttagtgtatcctcctttgatgtacttttaattttaatgtatttttattttatgtattgttaattttctttttaaattttagttttcacttttcaattttagcaacattagatatcttacatttgcatttttcatttttaaataattgttatatttctttttatacaattataataataataaaattaacttataattttatatataatatatataaaaattaatatatcaaaaaaataggatataaaattaaaattataaagatcttaatataaaaattaactatatacacaatatatgataaattaaagtccaaaaaaataaaaataaaaaagaataaaataataataaatcaaatttggtgttgatgaatagtgtcacaccaaatttggtgtgagactattcacatactaaaatggtgcaaaatttgatgttccattggagcaaaaaaaatactaaatcttacaccaaatttagatttgctgcaaaaaatagtgcatcattggagatgccctaagaccatctccaaggctgcattatagagcatgaatagtgttgcaccaaatttggtgcaacactattcatcactccatatttggtttattattattttattcaatctttttattttttggacttttaatttatcatatattgtgtatataattaatttttatattaagatctttataattttaattttatatcctattttttgatatattaattttgtatatattatatttatataaaattataagttaattttattattattataattgtataaaaagagatataaccgttatttaaaaataaaaaatgcaaatgtaagatatctaatgatgcgcatttcgcacttcgtaatgcattaatcgagcatttatgggagaataaaggcgtaagttaaatatttatgtggtacttaaattaaatttgactatgatgtaatatttatttaattatcttttatcaatgatttcacttttagttgatttatcctttaaaaaaattttgtaataaatgattatataagtggtgaatgttaattatatataatgaatatggaaaaaagaaaaaagatagtattagtttgaaggaaataaaaaatgaaaagtaaatagaagataataatataatatagaagagagagaagatttggtgtaaaaaattgtgtaatggttgaattaaatatggtgttacatcattttgatgtgaaatttggtgttagggttgcagatggcctaagaggagtgacctattgtctagatagtaataatgcagttttgtttaactaaagtagtggttatatgttcaactttagaggtttttgcttttacttgtatatatttttttcctggtgaataaacttttagttacccaaaaataataataattgagttaaaagaattgttacaaagaaacacaaataaggtaatattgtaaaccacgaagaaggtcagtgtgtgagatacaaaatgtcaggagaggtgtctgaaattattgtttttggcattgctgagaacattaacaataagaaaaaagcattaacaatcaacatatattcaaattggtaaaaaaacatgttcaaattggtgggttagaataagttaggacccattaactatttaatcagtttaaatttaggtagactctattatttgattgtagatataaaagataatattaaagagagaaactaccaacccctgtaacattaaaaaaaagttagaaacaatgttcattagaagatccaaaaggcaaaagataaaaataaagagaaataagatgaccgaaaccaacaattgatcgagcaaacaataaacaaagaggatagagaagaaaaactcacgaggaatcgagaaagacaaaggagaaggaaagagatatggaaaaatgaaaatcttagtttcagatggagtgctgaaggcaaaagggttaggaaaaattaaatcacgtgggaattggaagtgaataaatgtaaggccatagcacctcaaaatatacacgcagtcagaggctggacgggaccaggatttcaagtttatgggttcggaattccaatagtttgaagttactgtgttctagattaataatttatacatattcaatgatatttttaagacaaatatagtgttcgaaccaaagctactaggttcggccgaacccgctcccgccactatagctccacccttgcatgcagcaattaagtactccataatgattgaattacacataaacaaatgcataagcaacgtggtgtttgcaagtgaacagctgaaagtccatagcacctcaaaaaagactaaggtaagggtatcaatacaagcagcaattaagtaataaggaccaaatcacacagtatccctaaacaaatacttattaagtgatgaggtacgaatcggaatcgcacagtatcactaaacaaatgcatacaccacgtgggtgttatggaagtgaagtcataagcacctcaaaaatggaccaaattacacagttatccctaaacaaatgcataataccgaaactacccatgcacgaccataatacttcacttattatatagttatggcttctgcttccttggccaacaatcagttcatctctaacttcgaattccagttccattttcacttgacacacttcgaagcgccatctttgctactttaaggtaattgtatatttcaaaagtttgttttgcttatctgttttggaatgacagcggtaattgtgttgtttaacaaatttacatgctccaaatgaatggaagaagagttctaacttcaagaccatggccagaggccagttgttaattcctaagatcatcctgaacaaaatcttctctatatgtagcctctacgtactatattcgttcatgctttaatgtgtaatgcataacaagattttaccttaaatatccagatcgatcatatggcaactggtatcgcttcaggatgcggacagttacatttgaggaagcctgtctacttgaggaatagctatggaaataaagctcactctcattccaatgtgattctcaacggcacgcaaaaccagatcgcttggtacgttttaggggtaaaccagtaatatattttttcatgacgtgacacaattctagaagtagtcatttcctgattccttaggaaaagggaaggttatttcgtcccattttatatatcatagttacacattcttatatttaatagtaacaatttaactttaaaatacctcttttacccttaatgaaatgatttatagcgaaacacatatccattgctcagtttacaccataaatttcaaaaatattcttaaatattgtgttcagtcaaacatcatcacataaattgagacattgagacatagaggagtactatgttaattttctgatggtgatatgctttaccaggtctagttgggtttcaaatgtcttgcgagttaatagaagtagctatccacaatgtcaagtgataaaaacaaactggaagtctcggcgaggaacaatcaaatctagccagcagagagatggatcagttactaggtacttcgatttcattgtgattggtagtggaattgctggccttcgatatgcacttgaggttgccaagcatggaactgtggctgtgataaccaaggctgagccacatgagagtagcactaactatgctcaaggtggtgtaagtgctgtgctctgccctttggattcagtggagaaccacatacaagatacaattgtggcaggtgcttacctctgtgataaggagactgttaaagtaagttcacacgaatatatacagtttaatttggagactatttccccccttttgcttttgctataagtgtatctctcctttaatttctccaggtagtgtgtactgaaggacctgagagaattagagaactgatcgctataggtgcttcattcgatcatggggaggacggaaatctggatctagccagggaaggaggccactcccatcgtcgaattgtccatgctgctgatatgactggcagagagattgaaagagccttattagaggcagtgtttaagaatcctaatatacatgtgtttcaacaccattttgctatcgatttgttgaccactcaggttagtttattagtgtgctatagttgagtaaaggtcgcaattgaactattcagcaaggatttgatgttgtaatttgtatggcaaatgcaggatggttctgacgtagtatgtcatggcgttgatactatacacacggaaacgaaggaggtaagtaacagttgctttcactcatgttgacttttcaacattcttcaaaatgacataaattgattttcttacttgtgtattttaggttataagattcatttcaaaagtgactttgctagcatcaggtggagttggacatatctatccaagtactactaatccgacggtatggtttcaatatcttttcctccaaaatcttgttagttatgattaatgtcatgctccaaaaataaaagatctggacatggcactcgatcgatgctttgaaacttgtgacagagcgaaccaacatccattacatacttagtgcaattagaaatatgagctcgctgccctaaatgcctaaaaaaggattctgtttttatactttgaccatttgtgccaacagaaaagtttaaccctgttgaatgtgggcttgtttaactttctaattcatattgacattatgattataggttgcaactggtgatggaatggctatggctcatcgagctcaagctgtaatttccaacatggagtaagtaatcctcagtagcattatttttattgtacaatatctctgcctctgctttagtgagttttgtgctgtaaaatctgctgacctagatttcatcctttttttttttctttcctgatttctgcatcttgttcagcatttcgttcagaatttgcactttcgactaaaaacacaagggtgtgttcaaaaatttgcattattaataacaattctcttcctcgtgttgccaggtttgtgcaattccacccaactgccttggctgatgaagggcttcccaacataccaagtgccagagagaatgcttttttgataactgaagctgtcagaggtgatggaggcatcctttataacttagatatggaaagatttatgccaatgtatgatgaaagagcagaacttgccccgagagatgtggtagcaagaagtatagatgaccagctcaaaaagcgtggcgaaaagtatgttcttcttgatatcagtcacaagcccagagagaaggttctgtcccattttcctaatatagctgctgagtgtctccgccatgggttagacataacacagcagccgattccggtggttcctgctgctcactacatgtgtggtggagtccgtgctggactcgagggtgagactaatgtgcaaggtctttatgtggcaggtgaagttgcatgtactggtttacatggtgcaaaccgacttgctagcaactcattgcttgaagcactagtgtttgcacgaagagctgtacagccttcaattgatcatgtgaacgtgtctagaattgataacggtgcatcaagttggtggccgcggcctgtagcccccctggcactaggagatacagtacttaacaaagtcatccgtcggacaagggaagtgaggaaagaactacagtcaatcatgtgggaatatgttggaattgttaggtctacctcaagactaaatactgctgagaagagaatcaaagagttggagttggaatgggaaacatacctgtttcagcatggctgggaaccaacaatggttggagtagaggcttgtgagatgaggaatctcttctgttgtgccaacctggtagttagcagtgctctttctcgacaagagagtcgtgggcttcactacaccactgattttcctcatgttgaggaaagcgagaggttgccaacggttatctttccttctcagcgaaatagcacatggagcacacggcaattacacgcgcagccgataagttagatatctcttacctatttgccattcttcctgccaaaacatctccagtgcaggacatgatttgtcgattttaccgggttgcaggggtgtatctatcggaaggggtatgggttcatatgaacacatactcctctccatagactatgtataataatgtatatttcttcaatgttatttaaatatgcaagtgtgtcagccaagctcaaagagttcaataattattgggtacatctttacaagtgaaattgtgattttaaatcccatgtctattttgtcgtttttccctttatcttttccgccgaaagtcaaatctcacatttctcttgttggttttcctttcttttcctataaatgggtctacccatgataaaagaaatttcatatttttgttttagtaatttctgaatgcaggttttgacaatttattaaaaacatatcacaggtcacgagctttaattagttaagtaagcaacttgttaaatgtgccagacctgattcttagtgcaattcacccttcttcattttctaggatagttctcctagccagtctgtaacttgctctgttcatggcaaattacaagtgcgtgatagtttggagaccataggaaccctgaactcgaaattggggaaattagagaaaaggcatcgaaaattaaccataaatcagaacaaaatacctcaaaccatgagtacctccatgaattttgctctaaatcatgtaggttttgatcaaatttagctacaaacttgcgttctttggagagagagaattggaaagttaagtccattctagaagaaaatgacgaacatggtccctaatctattgggatttgatcattttggtccttaatgtatgcacttgacctatatagtccttaacctattttaaaaggtgactcttttggtttgaaacactataactaacggtatagttactagcacccactgggcatatggcttataagcatcaatagacgtagccttggaaaggaatggaaattttagggccttgtgagggtagagtaatccttggtaatggacatatttttcttttttataattaaatgatattactgaatggtattccaaacatgtcaattgttcctttttataaggcacataggtggggtaatccggaattgtatagtcgggtataacttctcgagtgatgagatgtttcagagtttaagtaattgaattctcatatatgggataagtattcactttagtgtaaatcttacttccagttaagacaggatattaagcgaccgaagaatacggccaaaagcgggggaagctagaagcgaaaaaatatctcgcttgagtcctccaaaggaagataagagatagtaatgttagtaagaaatagatagaaggataagtatgagaaatgtttaacaattataagctgaagtatggtattatgacaaggttcgtaatcaagaaaaagtgaaggcaagttttaattataaagaggtatgagtcgtaatcacgagaagtgaattttcgacttcaataagagttatcaaaagaccaatctagcccctggattaagaaataccaatattaggtagtaacctaagataacgagatgcaagttagaaactcaaaggatttctgtaatagttggcattgcgacatttacaaagtgaatgatcaggcagtaaaagggtgaatgactatggaacaacctttgagggttagtagaaagagctctccctgagagaagcgtcataagcaaagttaagctcatcaaggtcgagcataccagttatgagtatacaatactacatacatataagttatccaattgctttagtagggaagattaccccaaggcaagttataagccactgaaattgcaaagaattgcaaaaggtggagagttaacgatgtgacctctacaagagtggaattcaagagcataaggagttaattattctcccgagggaagatcgtatgataaagtatcgaggcaaaattatgaggttcgcttagtaacggagcggtaagaaggattacgacaagaggtttgaaaggaataagattgtacttacttagaccctacaaatgtgtaacgactctaatgcataagtacaaacggtagagaaaatgcagtaatgacttcctgactagaggtaccaattgatggtaaataaaactaggcagttgatactcaggaagctagtgtgaggggtaaattaaggcaaaaacatagcctcaagaggagttacttagattttacctatgaagataattgattgagcaatcagtgattagcttatgaagggtctagttatgggttagacgacaaaactcagacgagtcattagatcatgcaaaattacatgttggatcaaaacgtacaaagtttcagcctcgcaagtgcatgatcgcgactctcagaaagtatttcaagacataagcaatggtaggtgaaattccatattatcttttagaaaatcggaaggagcccattgagcttaaaatatgagggaggtgttcaaaagttgtgatcagaagtaatattatagtaaaggagaggtgaaaaacaattagatattattttagatagttcaaaatcacctaaagttctagggagtatatgatgtaatgagctcgcagtcagatatgaacaagagaatcttttctaagtgtgtatacgactaaaatcggagagtccgattttatgatcgttatgacattccacggctcagcttcagaaggcctgaggcacagttcgaagttcgaccccgagggttctcaatgcccaacctcggggtaacgtaaatcgacgactatcttgcataagcgaaaagttcccaaggcgcgtgctcaaagctgacaacacctgcaaatatagtataagttcgtactgtggcattaaatagctgtaccaggttcatatctttgtaataaatgcatatgtactatgttggggttctccctcctatataaaggggacccttgttatttttttcatacatgatatttaatacaaga

SEQ ID NO: 37 - DNA, 7038 bp, Nicotiana tabacum
cagatttggttaattttggtaagagtgaactcgtgagtgaatgggtgttcatatttggtaacttttacccgatttcgagacatggacccggggaggatttttaggacggatttcagattttttattaaaatcttgatttcattaattagattagtctattatagttgtatttatgatatgtaattaattttggctagatttgggccattcagagtcagatattcatgaaaaaggcattgttactgattgattgagcttggttcgaggtaagtggcttgcctaaccttgtgtgggggaactccccttaggatttggtactacttttgatatatgagctctgtgtatgtgaggtgacaagtgcgtacacgggctattattgcaaaactccattttcattaagtaatatacctgtcttcctttaactgagctacactagcatattaatttatcctgtttagtctagaacaacatgtctacgtgtcttaattgcttatgtgaactctgtgcatcatgcttagtaaattttctgcttctttcttgactgatacttagtctaaatcgtaagatttcgtgatgtagttgtatttctattgtttgcgctgtatatttactttgggactacagagcgatatttcggtagatcccccattctgcatatttactttgggattacggaacggtattccggtagatccctctgtcatgtatatttactttgggactacaaaacggtattccggtagatccccctgctctgcatatttactttgggactatagaacggtattccggtagatccccctgctctgcatatttactttgggactacggaacggtattccggtaaattccccctatttttgcacatttacatttgggactacgagacggtatcctgggagatcctctattgttatttctgtgtactgagttgttgacttgctatgatttcattcttgttaaatttcagtacttatttttactgcaatatttcattctgtcttagtttattatatatataccatgacctgatctcgtcactactcgaccgaggttaggcttggcacttattgggtaccgttgtggtatactcatgctactcttctgcacatattttttgtgtgcagatccaggtgctctttatcagtgagccgggacagctttggagacttcaaggtatatcttccgcgtccgcagacctcggagtccccttctactcttccccacgtccattatcttctgtattttccttttgttagactctgaagtatagagacactagattttccttctgttgtttgtaacttacgatattccgggttttgggagagttatgtacatttcgagagtgaccgtggtatatgccgagcgacatcttaatttcttatttagaatctacctgtaaattgctagttttaatgttttcgtttcatttccgcaaaagtgttaggcttacctagtcgtagagactaggtgtcgtcacgacggttcaagaagggagaacttgggtcgtgacaccttaatattattgtgccatttcgaaccaaaatattaagtaatttttattataattcaaactattaatagtaaatttatgttttttttgtatatataacaagaaaagagtaatctgatcaggaaaaaacatagattcaaattagaactcatgatattactgttcaaactgtaataactttaccatttgaatttttatgactattttgaatgtcaagtaaacatttcaaggtacaataaaaagaaagagcagacaattggtatcttctttagaaatatttgtttctatattttcaggtccacttctaatgtaacacatattttttcttatgttaaaagaagacatctcatcttatttaatactattaacaaatgaactatgaaaaatgcaaactctttgattgttcacaacttgacgaggtttaaataaattataatctttgtcttaaatatacgcgctaagaaactaccaaaatgtgttgcctatgaattttgtgctaccaaaaatagaatatgaggaaataacaactcacaaacacaaagaaaattaagttgatgaaatattgtccaccttttatttcttcttcattaatgtttaatcccaacaacataagtttaaaaccaaatgattaactcaaaaatgcaatagtttttattgaataaagatgcatatgaaatatccgtatttaaacatattatttaaattaactaaaagatctttgcaaaacaattggagtaatacaattaaggaaattatttttgtaataaaatgttgggacatgctcagcagcatggccagccctcctgtagtatacatatatgcagcaattaagtagtccttaatgattgaattacattacacctaaacaaatgcataaaccacgtggtatttgcaagtgaacagctgaaagtccatagcacctcaaaaaagactaaggtaacgtgggtatcaatatatgcagcaattaagtaataaggaccgaatcacatagtatccctaaacaaatataagtgatacatagtatcccctaaacaaatataagtgataaggtacgaatcactaaacaaatgcataaaccacgtgggcgtttggaagtgaagtcataagcacctctaaaattgatcaaattacacagttatccctaaacaaatgcataataccgaaactacccctgcacgaccataatacttcacttatatagttatggcttctgcttccttggccagcaatcatttcatctgtaacttcgaattccagttccattttcacttgatcgtacttcgaagcgccatattttcccctttaagctaaggtaattgtattgtttaacaaatttacatgttccaaatgaatattaattgttaattcctattatcatcctgaaacaaaattttctctatatgtagcctttacgtactatattcgctcatgctttaatgtgtaatgcataacaagattttaccttaaatatccagatcgatcatatggcaactggtatcgcttcaggatgcggacagttacacttgaggaagcctgtctacttgaggaatagctatggaaataaagctcactgtcattccaatgtgattctcaacggcacgcaaaaccagatcgcttggtacgttttaggggtaaaccagtaatatctttttcatgaaatgattaatagtcaaactattatccatggctcactttacgcaataaattttaaaagtattcttaaacatcgcgctaataatctgatggtgatatgcttttccaggtctagttgggtttcaaatgtcttgcgagttaatagaagtagctatccagaatgtcaagtgatcaagacaaactggaagtctagccgaggaacaatcaaatcgtgccagcagagagatggatcagttactaggtacttcgatttcactgtgattggtagtggaattgctggccttcgatatgcacttgaggttgccaagcatggaactgtggctgtaataaccaaggctgagccacatgagagtagcactaactatgctcaaggtggtgtaagtgctgtgctctgccctttggattcagtggagagccatatgcaagatacaattgtggcaggtgcttatctctgtgataaggagactgttagagtaagttcacacagaatatattcagtttggagactataaatttcccccttttgcctttactataagtgtatctctcctttaatttctccaggtagtgtgtactgaaggacctgagagaattagagaactgatcgctatgggtgcttcattcgatcatggggaggacggaaatctggatctagccagggaaggaggccactcccatcgtcgaattgtccatgctgctgatatgactggcagagagatagaaagagctctattagaggcagtttttaagaatcctaatatacatgtgtttcaacaccattttgctatagatttgttgaccactcaggttagtttattagtgtgaaaaaagtttttctatagttgtgtaaaggtggcaattgaactgttcagtaaggatttaatgttgtaatttgtatgccaaatgcaggatggttctgacatagtatgtcatggcgttgatactatacacacggaaacgaaggaggtaagcaccagttgctttcactcatgttgacttttgaacatttcttcaaaaggacacaaattgatttttatggcttctgcgctcttacttgtgttttttaggttataagattcatttcaaaagtgactttgctggcatcaggtggagttggacatatctatccaagtactactaatccgacggtatgggtttcaatatcttttcctacaaaatcttgttagttataattaatgtcacgctccaaaaataaatgagctggacatggcactcgaacgatgccttgaaactagtgacagagcgaaccaacatccattatatactccctgccctaaatgcctaaaaaaggattctgggtagtcgaataacagatgattctctgcctggaagtgtgaattcttattctatacacccataatttatgtacagtaaaagcaagatacatggttcaaagttttactaattacccgggtcaggcatctgctgtggctctgtaattggtggttgggtcaattctgtttttatactttgaccatttgtgccaacagaaaagtttaaccctgttgaatgtgggcttgtttaaatttctaattcatattgacattatgatcataggttgcaactggtgatggaatggctatggctcatcgagctcaagctgtaatttccaacatggagtaagtgatcctcagttgcattatttttattgtacaatatctctgcctctgctttagtgagttttgtgctgtaaaatctgctgatctagatttcatcctttttttccccctgatttctgcatcttgttcagcatttcgttcagaatttgcactttcgactaaaaacacaagggtgttaaaaaatttgcattattaataacgattctcttcctcgtgttgccaggtttgtgcaattccacccaactgccttggctgatgaaggccttcccaacataccaagtgccagagagaatgcttttttgataactgaagctgtcagaggtgatggaggcatcctttacaacttagatatggaaagatttatgccaatgtatgatgaaagagcagaacttgccccgagagatgtggtagcaagaagtatagatgaccagctcaaaaagcgtggcgaaaagtatgttcttcttgatatcagtcacaagcccagagagaaggttctttctcattttcctaatatagctgctgagtgtctccgccatgggttagacataacacagcagccgattccggtggttcctgctgctcactacatgtgtggtggagtccgtgctggactcgagggtgagactaatgtgcaaggtctttatgtggcaggtgaagttgcatgtactggtttacatggtgctaaccgacttgctagcaactcattgcttgaagcactagtgtttgcacgaagagctgtacagccttcaattgatcatgtgaacgtgtctagaattgatcacggtgcttcaagttggtggccgcggcctgtagcccccatggtactaggagatacagtacttaacaaagtcatctgtcggacaagggaagtgaggaaagaactacagtcaatcatgtgggaatatgttggaattgttaggtctaactcaagactaaacactgctgagaagagaatcagagagttggagttggaatgggaaacatacctatttcagcatggctgggaaccaacaatggttggagtagaggcttgtgagatgaggaatctcttctgttgtgccaacttggtagttagcagtgctctttctcgacatgagagtcgtgggcttcactacaccactgattttcctcatgttgaggaaagcgagaggttgccaacggtcatttttccttctcagcgaaataactcatggagctcacgccaattacacgcgcagccgataagttagatatctctttcctatttgccattcttcctgccaaaacatctccagtgcaggacatgatttgtcgattttaccgggttgcaggggtgtatctattggaaggggtatgtgttcacatgaacatatactcttttccctaaattatgtataataatatatatttcttcaatgttttttaagtatgtaagtgtgtcagtcaagctcaaagagttctatcgttcaataattattaggtgtatcttaacaagtaaaattgggattttaaatcccatgtctattttgtggtttttcccgttatcttttccgttgaaggttaaaatctcacatttctcttgttggtttttcctaaaaatgtgtctacccacgaggatgggcatgtcttgtgtctcctattgccttttagttaagtatttttttttcttgggaaaataacagttttagttaactatcaaagaagagataacaacttattacaaattatatgcgagaagcacggtgcctgtcatgcttcagaaagtcataatggcaaatcaaaattatcgccctcctaggtcaaacatcaatatggtttcattcttcttcttcacaaatccataagtcaatgacacacaataggttcattaatgattcagagaacatctaatccagcgaggggtcgtttggtttgaatacggcttatgacgggattaggtatgctaaaattagttatgttgggattagttatcctgatattattttttatccactgtttggtatgttaacgatcgggtacccctaagtaatttaatgaaaaggaatcaacaattgtttcaacaagaacaaaacacctattggtgcttgagaaaatatagatgtctcgggcattaaatccatgataaaggctaatgcgtacctcaatcttttagctcttccattacttaaaagagtttccccctactgtacaaagtaaatgaggggaataaagaaatccataaaagaaatttcctatttatggtttagtaat

SEQ ID NO: 38 - DNA, 18 bp, Artificial Sequence
  Synthetic Primer
gctgctgagtgtctccgc

SEQ ID NO: 39 - DNA, 21 bp, Artificial Sequence
  Synthetic Primer
tccaccacacatgtagtgagc

SEQ ID NO: 40 - DNA, 30 bp, Artificial Sequence
  Synthetic Probe
tgggttagacataacacagcagccgattcc

SEQ ID NO: 41 - DNA, 23 bp, Artificial Sequence
  Synthetic Primer
gaggttgccaacaatcatttttc

SEQ ID NO: 42 - DNA, 21 bp, Artificial Sequence
  Synthetic Primer
tgcgcttgacaagttttagca

SEQ ID NO: 43 - DNA, 29 bp, Artificial Sequence
  Synthetic Probe
ctcacggcaattacacaggcagcagatat

SEQ ID NO: 44 - DNA, 29 bp, Artificial Sequence
  Synthetic Primer
agatatctcttacctatttgccattcttc

SEQ ID NO: 45 - DNA, 24 bp, Artificial Sequence
  Synthetic Primer
ccataccccttccgatagatacac

SEQ ID NO: 46 - DNA, 26 bp, Artificial Sequence
  Synthetic Probe
tgccaaaacatctccagtgcaggaca

SEQ ID NO: 47 - DNA, 20 bp, Artificial Sequence
  Synthetic Primer
ctaagggtgctgccagcttt

SEQ ID NO: 48 - DNA, 22 bp, Artificial Sequence
  Synthetic Primer
gtcaagcactggagcatatcca

SEQ ID NO: 49 - DNA, 26 bp, Artificial Sequence
  Synthetic Probe
atcatgaaccatccaggacagattgg

SEQ ID NO: 50 - DNA, 30 bp, Artificial Sequence
  Synthetic Primer
taagagacagacctcagaattgggtgtgcc

SEQ ID NO: 51 - DNA, 30 bp, Artificial Sequence
  Synthetic Primer
taagagacaggatagagaggagagataggc

SEQ ID NO: 52 - DNA, 30 bp, Artificial Sequence
  Synthetic Primer
taagagacagatgctctagaagttgcaaag

SEQ ID NO: 53 - DNA, 29 bp, Artificial Sequence
  Synthetic Primer
taagagacagttctcccgtgccttctcac

SEQ ID NO: 54 - DNA, 30 bp, Artificial Sequence
  Synthetic Primer
taagagacagttttccatgtaaacatttgc

SEQ ID NO: 55 - DNA, 30 bp, Artificial Sequence
  Synthetic Primer
taagagacagtgacatccctcataaatgaa

SEQ ID NO: 56 - DNA, 30 bp, Artificial Sequence
  Synthetic Primer
taagagacaggggagtgctaatctgatatg

SEQ ID NO: 57 - DNA, 32 bp, Artificial Sequence
  Synthetic Primer
taagagacagggcaatagaaagaagataatac

SEQ ID NO: 58 - DNA, 30 bp, Artificial Sequence
  Synthetic Primer
taagagacagttattcctccaatgagaacg

SEQ ID NO: 59 - DNA, 30 bp, Artificial Sequence
  Synthetic Primer
taagagacagtaccaatcaccgcgaaatcg

SEQ ID NO: 60 - DNA, 31 bp, Artificial Sequence
  Synthetic Primer
taagagacaggtttagtatactcttttgaag

SEQ ID NO: 61 - DNA, 30 bp, Artificial Sequence
  Synthetic Primer
taagagacagctatagcaaaattttcacac

SEQ ID NO: 62 - protein, 644 aa, Nicotiana sylvestris
MATGIASGSGQLHLRKPVYWRSSYGKAHCHSNAILNGMQNQIPWSYWVSKFLRVHRSNYSQCQVKTNWKSHTGTINSCQRDGSTRYFDFAVIGSGIAGLRYALEVAKHGTVAVITKAEPHESNTNYAQGGVSAVFCPMDSVESHMQDTIVAGAYLCDEETVRVVCTEGPERIRELIAMGASFDHGEDGNLHLAREGGHSHRRIVHAADMTGREIERALLEAVFKHPNIHVFQHHFAIDFLTTQDRSDIICHGVDAINTETQEVIRFISKVTLLASGGAGHIYPSTTNPPVATGDGMAMAHRAQAVISNMEFVQFHPTALADEGLPNRPSARENAFLITEAVRGDGGILYNLDMERFMPMYDKRAELAPRDVVARSIDDQLKKRGEKYVLLDISHKPREKVLSHFPNIAAECLRHGLDITQQPIPVVPAAHYMCGGVRAGLEGETNVQGLYVAGEVACTGLHGANRLASNSLLEALVFARRAVQPSIDHVNVSRIDHCASSWWPRPVAPVVIGDTVLNKVIRRTREVRKELQSIMWEYVGIVRSTSRLTAAEKRINELELEWETYLFQHGWEPTMVGLEACEMRNLFCCANLVVSSALSRHESRGLHYTIDFPHVVESKRLPTIIFPSQRNSSWSSRQLHRQQIC

SEQ ID NO: 63 - protein, 644 aa, Nicotiana tabacum
MATGIASGSGQLHLRKPVYWRSSYGKAHCHSNAILNGMQNQIPWSYWVSKFLRVHRSNYSQCQVKTNWKSHTGTINSCQRDGSTRYFDFAVIGSGIAGLRYALEVAKHGTVAVITKAEPHESNTNYAQGGVSAVFCPMDSVESHMQDTIVAGAYLCDEETVRVVCTEGPERIRELIAMGASFDHGEDGNLHLAREGGHSHRRIVHAADMTGREIERALLEAVFKHPNIHVFQHHFAIDFLTTQDGSDIICHGVDAINTETQEVIRFISKVTLLASGGAGHIYPSTTNPPVATGDGMAMAHRAQAVISNMEFVQFHPTALADEGLPNRPSARENAFLITEAVRGDGGILYNLDMERFMPMYDKRAELAPRDVVARSIDDQLKKRGEKYVLLDISHKPREKVLSHFPNIAAECLRHGLDITQQPIPVVPAAHYMCGGVRAGLEGETNVQGLYVAGEVACTGLHGANRLASNSLLEALVFARRAVQPSIDHVNVSRIDHCASSWWPRPVAPVVIGDTVLNKVIRRTREVRKELQSIMWEYVGIVRSTSRLTAAEKRINELELEWETYLFQHGWEPTMVGLEACEMRNLFCCANLVVSSALSRHESRGLHYTIDFPHVVESKRLPTIIFPSQRNSSWSSRQLHRQQIC

SEQ ID NO: 64 - protein, 645 aa, Nicotiana tabacum
MATGIASVSGQLHLRKPVYWRSSYGKAQCHSNVILNGMQNQIPWSYWVSKFLRVHRSNYSQCQVKTNWKSHSGTINSCQRDGSTRYFDFAVIGSGIAGLRYALEVAKHGTVAVITKAEPHESNTNYAQGGVSAVLCPMDSVESHMQDTIVAGAYLCDEETVRVVCTEGPERIKELIAMGASFDHGEDGNLHLAREGGHSHRRIVHAADMTGREIERALLEAVFKHPNIHVFQHHFAIDLLTTQDGSDIVCHGVDTINTETQEVIRFISKVTLLASGGAGHTYPSTTNPPVATGDGMAMAHRAQAVISNMEFVQFHPTALADEGLPIRPTRTRENAFLITEAVRGDGGILYNLDMERFMPMYDERAELAPRDVVARSIDDQLKKRGEKYVLLDISYKPREKVLSHFPNIAAECLRHGLDITQQPIPVVPAAHYMCGGVRAGLEGETNVHGLYVAGEVACTGLHGANRLASNSLLEALVFARRAVQPSIDHMNVSRIDHGASSWWSRPVAPMLLGDTVHGKVIHRTREVRKELQSIMWEYVGIVRSTSRLTAAEKRIRELELEWETYLFQHGWEPTMVGVEACEMRNLFCCANLVVNSALSRHESRGLHYTIDFPHVEESKRLPTIIFPSQRNSSWSSRQLHRQQIC

SEQ ID NO: 65 - DNA, 1935 bp, Nicotiana sylvestris
atggcaactggtatcgcttcaggaagcggacagttacatttgaggaagcctgtctactggaggagtagctatggaaaagctcactgtcattccaatgcgatcctgaatggcatgcaaaaccagatcccttggtcttattgggtttccaaattcttgcgagttcatagaagtaactactcacaatgtcaagtgaaaacaaactggaagtctcacaccggaacaatcaattcttgccagagagatggctcaactaggtattttgattttgctgtgattggtagtggaattgctggccttagatatgctctagaagttgcaaagcatggaactgtagctgtgataaccaaggctgagcctcatgagagtaacactaactatgctcaaggtggtgtaagtgctgtgttctgccctatggattcagtggagagccacatgcaagacacaattgtggcaggtgcttacctctgtgatgaggagactgttagagttgtgtgtaccgaaggacctgagagaattagagaactgattgctatgggtgcttcattcgatcatggggaggacgggaatctgcatctagccagggaagggggccactcccatcgtcgaattgtccatgctgctgatatgactggcagagagatagaaagggccctattagaggcagtttttaagcatcctaatatacatgtgtttcaacaccattttgctatagattttttgaccactcaggatcgttctgacataatatgtcatggcgttgatgctataaacacggaaacgcaggaagttataagattcatttcaaaagtgactttgctggcatcaggtggagctgggcatatctatccaagtactactaatccaccggttgcaactggagatggaatggctatggctcatcgagctcaagctgtaatttccaacatggagtttgtgcaattccatccaactgccttggctgatgaaggccttcccaacagaccaagtgccagagagaatgcttttttgataactgaagctgtcagaggtgatggaggcatcctttacaacttagatatggagagatttatgccaatgtatgacaaaagagcagagcttgccccgagagatgtggtagcaagaagtatagatgaccagctcaaaaagcgtggcgaaaagtatgttcttcttgatatcagtcacaagcccagagagaaggttctgtctcattttcctaatatagctgctgagtgtctccgccatgggttagacataacacagcagccgattccggtggttcctgctgctcactacatgtgtggtggagttcgtgctggacttgagggtgagactaatgtgcaaggcctttatgtggcaggtgaagttgcatgtactggtttacatggtgctaaccgacttgctagcaactcgttgcttgaagcactagtgtttgcacgaagagctgtacaaccttcaattgatcacgtgaatgtgtctagaattgatcactgtgcttcaagttggtggccgcgacctgtagccccagtggtaataggagatacagtacttaacaaagtcattcgtcggacaagggaagtgaggaaagaactacagtcaatcatgtgggaatatgttggaattgttaggtctacctcaagactaaccgcagctgagaagagaatcaatgagttggagttggaatgggaaacatacctatttcagcatggctgggaaccaacaatggttggactagaggcttgtgagatgaggaatctcttctgttgtgccaacctggtagttagcagtgctctttctcgacacgagagtcgcgggcttcattacaccattgattttcctcatgttgtggaaagcaagaggttgccaacaatcatttttccttcacagcgaaatagctcgtggagctcacggcaattacacaggcagcagatatgttag

SEQ ID NO: 66 - DNA, 1935 bp, Nicotiana tabacum
atggcaactggtatcgcttcaggaagcggacagttacatttgaggaagcctgtctactggaggagtagctatggaaaagctcactgtcattccaatgcgatcctgaatggcatgcaaaaccagatcccttggtcttattgggtttccaaattcttgcgagttcatagaagtaactactcacaatgtcaagtgaaaacaaactggaagtctcacaccggaacaatcaattcttgccagagagatggctcaactaggtattttgattttgctgtgattggtagtggaattgctggccttagatatgctctagaagttgcaaagcatggaactgtagctgtgataaccaaggctgagcctcatgagagtaacactaactatgctcaaggtggtgtaagtgctgtgttctgccctatggattcagtggagagccacatgcaagacacaattgtggcaggtgcttacctctgtgatgaggagactgttagagttgtgtgtaccgaaggacctgagagaattagagaactgattgctatgggtgcttcattcgatcatggggaggacgggaatctgcatctagccagggaagggggccactcccatcgtcgaattgtccatgctgctgatatgactggcagagagatagaaagggccctattagaggcagtttttaagcatcctaatatacatgtgtttcaacaccattttgctatagattttttgaccactcaggatggttctgacataatatgtcatggcgttgatgctataaacacggaaacgcaggaagttataagattcatttcaaaagtgactttgctggcatcaggtggagctgggcatatctatccaagtactactaatccaccggttgcaactggagatggaatggctatggctcatcgagctcaagctgtaatttccaacatggagtttgtgcaattccatccaactgccttggctgatgaaggccttcccaacagaccaagtgccagagagaatgcttttttgataactgaagctgtcagaggtgatggaggcatcctttacaacttagatatggagagatttatgccaatgtatgacaaaagagcagagcttgccccgagagatgtggtagcaagaagtatagatgaccagctcaaaaagcgtggcgaaaagtatgttcttcttgatatcagtcacaagcccagagagaaggttctgtctcattttcctaatatagctgctgagtgtctccgccatgggttagacataacacagcagccgattccggtggttcctgctgctcactacatgtgtggtggagttcgtgctggacttgagggtgagactaatgtgcaaggcctttatgtggcaggtgaagttgcatgtactggtttacatggtgctaaccgacttgctagcaactcgttgcttgaagcactagtgtttgcacgaagagctgtacaaccttcaattgatcacgtgaatgtgtctagaattgatcactgtgcttcaagttggtggccgcgacctgtagccccagtggtaataggagatacagtacttaacaaagtcattcgtcggacaagggaagtgaggaaagaactacagtcaatcatgtgggaatatgttggaattgttaggtctacctcaagactaaccgcagctgagaagagaatcaatgagttggagttggaatgggaaacatacctatttcagcatggctgggaaccaacaatggttggactagaggcttgtgagatgaggaatctcttctgttgtgccaacctggtagttagcagtgctctttctcgacacgagagtcgcgggcttcattacaccattgattttcctcatgttgtggaaagcaagaggttgccaacaatcatttttccttcacagcgaaatagctcgtggagctcacggcaattacacaggcagcagatatgttag

SEQ ID NO: 67 - DNA, 1938 bp, Nicotiana tabacum
atggcaactggtatcgcttcagtaagcggacagttacatttgaggaagcctgtctactggaggagtagctatggaaaagctcagtgtcattccaatgtgatcctgaatggcatgcaaaaccagatcccttggtcttattgggtttccaaattcttgcgagttcatagaagtaactattcacaatgtcaagtgaaaacaaactggaagtctcacagcggaacaatcaattcttgccagagagatggctcaactaggtatttcgatttcgcggtgattggtagtggaattgctggccttcgatatgctcttgaagttgccaaacatggaactgtagctgtgataaccaaagctgagccacatgagagtaacactaactatgctcaaggtggtgtaagtgctgtgctctgccctatggattcagtggagagccacatgcaagatacaattgttgcaggtgcttacctctgtgatgaggagactgttagagttgtgtgtaccgaaggacctgagagaattaaagaactgattgctatgggtgcttcattcgatcatggggaggatggaaatctgcatctagccagggaagggggccactcccatcgtcgaattgtccatgctgctgatatgactggcagagagatagaaagggccctattagaggcagtttttaagcatcctaatatacatgtgtttcaacaccattttgctatagatttgttgaccactcaggatggttctgacatagtatgtcatggcgttgatactataaacacggaaacacaggaggttataagattcatttcaaaagtgactttgctggcatcaggtggagctgggcatacctatcctagtactactaatccgccggttgcaactggagatggaatggctatggctcatcgagctcaagctgtaatttctaacatggagtttgtgcaattccacccaaccgctttggctgatgaaggccttcccatcagaccaacaagaaccagagagaacgcttttttgataactgaagctgtcagaggtgatggaggcatcctttacaacttagatatggagagatttatgccaatgtatgatgaaagagcagagcttgccccgagagatgtggtagcaagaagtatagatgaccagctcaaaaagcgtggtgaaaagtatgttcttcttgatatcagttacaagccccgagagaaggttctttctcattttcctaatatagctgctgagtgtctccgccatgggttagacataacacagcagccgattccagtggttcctgctgctcactacatgtgtggtggagtccgtgctggactcgagggtgagactaacgtgcatggtctttatgtggcaggtgaagttgcatgtactggtttacatggtgcgaaccgacttgctagcaactcgttgcttgaagcactagtgtttgcacgaagagctgtacagccttcaattgatcacatgaatgtgtctagaattgatcacggtgcttcaagttggtggtcgcggcctgtagctcccatgttactaggagatacagtacatggcaaagtcattcaccggacaagggaagtaaggaaagaactgcagtcaatcatgtgggaatatgttggaattgttaggtctacctcaagactaaccgcagctgagaagagaatcagagagttggagttggaatgggaaacatacctatttcagcatggctgggaaccaacaatggttggagtagaggcttgtgagatgaggaatctcttctgttgtgccaacctggtagttaacagtgctctttctcgacacgagagtcgcggtcttcattacaccattgattttcctcatgttgaggaaagcaaaaggttgccaacgatcatttttccgtcacagcgaaatagctcatggagctcgcggcaattacacaggcagcagatatgttag

SEQ ID NO: 68 - DNA, 23225 bp, Nicotiana sylvestris
gcttccttggccaacaatcagttaatttgtaacttcgaattcgagttcaattctacttcggagcgccatttttgccccgttaaggtaactgtattgttcaaaactttttttgttttgtcgatctatttttttttgttttgttttggaataataactatagttgtaattttttgggtgggggatgtggttgtaatttagtctagggttctgttaggttggggatgctagaatcttgagaagctttataaatatacgaacatgcagttgtatgataaactgatagccggtagatcctgttgttgcgaacatgctatgctagctcaattctgctctctgttccctttttctactgttttctttccctggtaaagcaacacaggctgacacaatcctagcccaaatgagagtaacaaagtttccagtctttagaaggtgaaatctataagcaaatagatgtgaatgtaagtgccttctggggcatacgattaacaaatagacgtgaatttaaatcactgcaggaattgagagaagaaatatagagtgtgttcggtataactgaaaatgttttcacttattctccagtatttggctggtgagggcaaaatatttccggagaatatttacaaatgtttgtttggtgagtggaaattgtttcctaatgttgttacaaaataattttctttttgatttcatttaggccccttaaagttcttgaaagattaactgcagaaaaaagtattcaacatgacatgtcattcttgtaagaacaagtcattaagaaaaagaaaaataatatattaaaattagaaagtttctaaatatatgaaaatgtcaatcttttgtaaataattcaagaaaatgaataatgacagtaatttaaaagtatcacagatttacataaagaaaggaaaaggaaaagagagaatggtacatgaaattttaaatgctttggctagattcaaattccatactcctattaaaagaaatgcctgacaggtaagaacatataggtactgttgtgtcaacatgcaatagcatttggtcactttggagagagtatagagaaaaagagaaaatggcagagggaagtgggagggaggcaagagccgattgtctagcgccaaaaagtttgatatgttctggatattggaaattgactttccttgggttcttaggtaagttagtttcatcaaaattaaaggaaaatgttttctttaggaaaatgtttccccaacaatttaggccaaccaaacatggtaaaattggaaaagattatcaagaaaatgttttctttcataccaaatacacccataagtaggagggattgtgataaattttgcaagttgtttatgtattttcagagatctatttacctgtcatacatgttctacaaaacacgagtccatgtatatatcattgcacttctcctttacaacttatttaatttctatttaaacagctttagcgcgtaagagctgttcatttccttgaacaccattgccaaagaacggtttaatgagggaaaatgaaaatttagctatgttggcaagtcctgagtcttagagcaaatgatcttcattgggtcttattgtttccttgcaatacttgttcagtcttgtaagttctgattttcgctaaaacaactctttttagtcgtcacttgttacttacaatttcctttctcctaatagaaacgtgtccggaaagctgacttttggccctgtatgtgtttctggtttttggagccttcagaatgatagtactagctgttcaggtgtctattgagggtcttcatcaaagcaacagtaaggaaatagttagaaaaactgaaaaggacttctccttaacgtgtttcagtctcttgattttaaaggaaatgcattttgtagatacattggcattcattgaaaatggccttgactcaatacctatgtcatgtgacatcaggaagggaaagcaatgatttctctttctgtttcagtaataagtgatgaagtcttgtggcaacttccatttgtaaattcattttgtacaagtggattatagaaaattagttgataagttcatacctttcttttctctactttttctcttgcaatatgagatatcacaggttagagacatgatgcacattcatttgtggttcacttgaatgagaaaaaagtatatgtttcttctttttatgtttcgtttccttttggttttcagtatctggtatcgaagttgtgtaataaacagtttgttccacgcatgtgctgctgcagcattaacatggactagccatcttgtcgtaggagttcaatttgtggaattccggtttaagcccatcaactgtggaatctctaaatattttcattgaattcaccatacgttagatgatatgttttctcatggtcctttcaagcacttctccttctgtttaaatgtctccacatgcttttctgccccttcaatatcagaatttgtctaaaagttcctttttctttaataaatctactgctccaaatgaatgatagaagagttgtaaagagttctgacttcaagaccaagcacagttttggttgggctttcaaattagcttataggaagttgttcctaagatcgtcctgaaacaaaatcttttctttttgtagcttctactgtattcattcatgctttaatgcaatttataacaaggtttcccctaaatatccagagtctttaattttgctttcgagtcccagctgcgcaaaacgtattaccgaagaatagttttctgggagatgttacaagagtttggttagaagggtctttcccttctaaagtgtttggttcaagttatctaaatgtcaagagccaatattttgttattaagctcaattccttgccctgtttgggtgtttttagaggtaatcaagatgatttttaaatgtttagtttcactaacattctaacctcagaattgggtgtgccaatctgatatcaattcctttgacttggattgtcagtcaggaagatcatatggcaactggtatcgcttcaggaagcggacagttacatttgaggaagcctgtctactggaggagtagctatggaaaagctcactgtcattccaatgcgatcctgaatggcatgcaaaaccagatcccttggtccgtattaggatgatgtttcttcgcctatctctcctctctatctttccctgctttattatcttcattctattgccccttctcctctcttttgggggaataattgtcaaaatgttttattttggagctttcaagatgttattacattccaatttgtacggacataggcattcacgtgttggctgttggactgtttattcctcccatgagaacttactggaaagaatctttgtatacgtgtttaggcataaaccagtaatatcttttttcatgagataccagaatcctaaaagttttttttttgagtcatttcctgattctttaggaaaaaaagaaaggttatcattttcattttctggtggtgatatgctacttaaattttccaggtcttattgggtttccaaattcttgcgagttcatagaagtaactactcacaatgtcaagtgaaaacaaactggaagtctcacaccggaacaatcaattcttgccagagagatggctcaactaggtattttgattttgctgtgattggtagtggaattgctggccttagatatgctctagaagttgcaaagcatggaactgtagctgtgataaccaaggctgagcctcatgagagtaacactaactatgctcaaggtggtgtaagtgctgtgttctgccctatggattcagtggagagccacatgcaagacacaattgtggcaggtgcttacctctgtgatgaggagactgttagagtaagttcacagaatattattgtctcttcagttccgtgaagcagtttgccctttttcagttttttctctttggaagctgtttcctttgcttttccaaatttttccaggactgcttggttggatgaataggaaagttctccatctttcaggttgaaacgaaaggaactttctgtttagacggcttttgccacaggatctagaactgccaaaaaatggaaaagggtaagagcaatcgggcagttaggcttgttttcaattagaagctgaagagccaagcaataatactaaagaaaggctctatgcctattccttccttctgatgtaagtgcttacaagttggaaccgaagaaagagttggagagttgagaaaccaatggttggtaatatggacgacttcctctggtttatgtagtgctcctattcttcatggttcagattgttgaatttgtctttgaacatcgtgagaaggcacgggagaaaatatgattgatattattctcatatgttaaacatgatacaatgagccctgtatatacataacatgtcctactcctaatacatatgggattagggttacataactattctaacactcccctcaagctggtgcatataaatcatatgtaccgagcttgttacatatgtagttaatacgaggaccagtgagagacttggtgaaaatatctgcaagctgatcattcgacttcacaaactttgtagcaatatctcccgagagtatcttttctctgacaaaatgacagtcaatctcaatgtgtttagttctctcatgaaacactggatttgatgcaatatgaagagcagcttgattatcacacacaagtcccatctgactaatctcaccaaatttcaactccttgagcaactgtttgatccaaattagctcacatgtcaccatagccattgctcgatattctgcttttgcactagaccgagcaaccacattctgtttcttgctcttccaagataccaaatttcctcctactaagacacaatatccagaaatagaacgtctatcagaaggtgatcctgcccaatcagcatctgagtatccaacgatctgctcatggcctcgatcctcaaacaataaacctttgcctgaagctgattttatataccgaagaatacgaacaactgcatcccaatgactatcacacggagaatccataaactgactcacaacactcacaggaaaggaaatgtcaggtcttgtcactgtaaggtaatttaatttaccaaccaaccgcctatatattgtaggattgctaagaggctccccctgtcctggcagaagtttagaattcggatccatcggagtgtcaacaggtctacaacctgtcattcctgtctcctcaagaatatctaaggcatacttccgttgtgagatcacaatatctgagctagactgagcgatctcaatacctagaaaatactttagtttgcccagttccttagtttgaaagcgttgaaagagatgttgcttcaatttagtaataccatcctggtcattgccggtaataacaatattgtcaacatagaccaccggataaatatagagactcgaagcaaaatgccgatagaatacagagtgatcagcttcactccgagtcatgccaaattcctggataactatgctgaacttaccaaatcaggctcgaggagattgctttagaccataaagtaatcggcgcaagtgacatactaggccacgagactccccctgagcaacaaacctaggtggttgctccatataaacttcatcctcaaggtcaccgtgtaaaaaaacattcttaatgtccagctgatagagtggccaatggcgaacaacaaccatggatagaaaaaggcggactgatgctatcttagccacgggagagaaggtatcactgtaatcaagcccaaatatctgagtatatcccttggcaacaagacgagccttaagacgatcaaccttaccatccggatcaaccttgactgcatacacccaacgacaaccaacactagatttacctgaaggaagagggacaagctcccaagtaccactcgtatgtaaatcagacatctcgtcaatcctgtcgccatcctggatgagacaatgcttcacctgtagacttagggatggaaacagaggacaaagaagatagaaaagcataatagggtgaagacaaacgatgataacttaaaccgacataatggggattaggattaagggtggtccgtatacctttccgaagtgcaatcgatgtactaggaagagacaagtccgcagtaggaccagggtcaggtgcaggacgtgaatcagctgggcctgatgctgggtgcagatgacgatggtatgtcaagagtggtgttcctgtggcagggagtgtaagaggagccacactagactccccaacggttggaatgggtaagacttctgtggcggaaggtgaagaaggagatatagtagaatccttaaaggtcggtataggtaagacctcagatatatcaaggtggtcagaagaggtaaagaaaggtttagactcaaaaaatgtgacgtcggaggacataaagtacctacgaagatcaagtgaataacaacgatatcccttctgaacacgagaataaccaaggaagacacacttgagagcacgaggagctaacttatctttcccaggggctaagttatgaacgaaacaagtgctcccaaaaacacgagggggaacagagtataagggtgacgggggaaacaatactgcatacaaaatctgattctggatgggagatgaaggcatccaattaaccaaataacaagctgtgagaactgcatcgccccaaaaacgcaacggaacatgagattcaataagaagtgtgtgagcagtctcaatgatgtgcctattctttctatctgcaaccctattttgctgaggggtataaggacaagaggtctgatgaataatttcttgagaagtcataaactggtaaaattgagaggataaatactctaaggcattatcactgcgaaaagtgcgaataaaaacacgaaattgatttttaatttcagcacaaaaattctggaatatagaaaacaactcagaacgatctttcattaagaaaatccaagtacatcttgaatgatcatcaataaaactaacaaaataacgaaatcccaaggttgaattgactctactaggaccccatatatcagaatgaactaaagaaaaaatagactctgcatgactctcaatactacggggaaaggaggctcaggtatgtttctcgagctgacatgactctcattctaatgtagataaactagacaaactaggcaccatcttctgaagcttggataaacttggatgtcctaaatgtctgcgaattaggtctggaggatctgtaactagacatgccttggaggaattgagtgagttaaggtagtaaaggccttctgattcaagtcttgttccaatcgtctgtcccgtactgcggtcctgcataataaaagaatcatcaataaaatatataccccaatggagggcacgagtcaaatgactaacagatgtaagattaaaaggacaaccagggacataaagaacggaatctagagtgacagagggtaggggattcgcttgtccaacaccttttactttagtttgagacccattggctaaagtaacagtgggaagagactgtgaatacgcaatatttgacaaaagtgatttattaccaaaaatatgatcagaagcggctgagtccacaatccattgtccaagagtactagactgggaaacacaagcaaaagaattaccagcaacagaagtatcagtctgagcaatagaggctacttgtggagatgtttgcttatttgctcgatattgaaggaactcattatactccccttcagataaagaaaatccctggttacctgtagtctcggtctgagcaacataagcatttttgggtgggcgaccatgtaaagaatagcacacgttactagtgtgtccaagtttatgacaataagagcacttgagtctagatttccaaaacgacctcctcctcgtctattctccatagtttgagatgcccgattgtccactgactgggatacgaggacagatgagtcaagtgtctgtgatgagctcactgggtgacttggtgctgcagcaaggcgaagtaatcgagagaataattcatcaactgtggggacagtcggtctagccaaaatctggtcacatactgaatcaaggtcattagggagtccagcgagtgtaagaactacaatatcctctgtcgttgctcttgttgcttttcaatactagcagaaactggcatcaacgtctcaaattcttccatgactgcctgtacttgttccaagtaagtagatatatccaattcctgtttcttcaagcttgtcattcgcaatattacatcatagagacgagatatgtcattagtgtataaattacgagccttttcccaaactaaataacatgtatggaatggacggaacaagagcatcaatttggaatcaatagatcgccacaagatactacataactgagcattgaccttctcccaaagtgttttggccttttcatcaccttcgctagccttttttgttaaatgatcttgaactcgttgacctttacaccacaactcgaaagacgaagcccaagctaagtagtttgaacctcccattaaaggttctgaggtaatcgtaacaccggaattgccagaacccgggtttttagacccgaaagcatcgactcccaaagacatcgttggattatcaccaaataacagaaagaatcaactgacaacttgctgaaacaggtgaaggaaacactgtttttgccggaaaattactgtagctgccggaaaaagtcggtgtagtcgccggaaaaactcaaagtggtcggaatcaaacgaaaaaggtatggagactcggaattactaggcgatccgactgtccaactggaagtttttcaaaaaaatggttggaacagtgctcacgcgccagtgcgtggggcgcttgggtcagatctcgccagaaagtttttggcgcgtgagggcgcgtgtacgtgagttttccggtggggtttactagggtttggtcgccggagcctgaggagtcttgtggtgttattggttttttgcacacaccaacaaaaattgatgtgattacgagcagccttctaagtcgccgtaaaattgcacggcgacgaggtctttcttcccggaagtcgctggaatgatgcacaacgataggtttctcactaaagctctgataccatgtgagaaggcacgggagaaaatatgattgatattaaacatgatacaatgagccctatatatacataacatgtcctactcctaatacatatgggattagggttacataactattctaacaaacattatgaaaagagagtgaaggtgacatgcaggaaggaagagataaggataagacaggaaattcacatgtgttgtcttttggttttattttgggatttcatttagtttgtgccacagtaccatgtttttttttcttaatgagaacacacttctgacttccctaaatcagcaccaattttctgagggtaactgctgataaggatagacactccaaggttatccaggattcctagcttaagttgtatcatataagtttctctcctatcccctcaagagtcctatgtacagaaaactctatcccttctctctcgagctttagctccggagtccatttacttttgttaatgctaacaactcttgcggagttgtgaagtgccttcttctgccgagagtagtaaggcccaatggacttcgcatctagtaggcccattatcaacatacaatgagggagaagggatagagttctctgtatataactcttgtggggataagagagaatcttatatgatacaacttaagctaggtgttagcggaaacgtaaaagaaagaacacaagatttaacgtggttcggatcaaaataatcctacgtccaccagagaacaattgcccttttaatattaacaaaggaaggggagatttcccaattacacttaagagaatttctctcttaactctctactcactacaatgtattgtattattttgggatgatttctacaagtgaaggagtgcatctatttatataggtaaagatgacatcaagaggaggtagtttgatgtcatgggtgacatcaaaggaggaagcttcctcctagcatccacaccaactctttccaccaactcttccaattggcatgccattgttgactaaacataaaccaacattttcagcatgccattgttaactaaacataaaccaacattttcactagggatcctggattgccttggagtgtctatccttatcaaccgcttagtttgctgtatactattttcatttgtctctgtaaatatatactggtttcaaggaagttttgtgttgtgcttggtagatgggatatcacaactaatatcttcttatcagttgataaaatcctggtccatgtaattctgctttttatgcaatctatgttctaaatgaaatttatgagatggctgatttattactccaaaattgtgtttagtctactcttttaaaatcttcgtttttataagtatatctcctttctccaggttgtgtgtaccgaaggacctgagagaattagagaactgattgctatgggtgcttcattcgatcatggggaggacgggaatctgcatctagccagggaagggggccactcccatcgtcgaattgtccatgctgctgatatgactggcagagagatagaaagggccctattagaggcagtttttaagcatcctaatatacatgtgtttcaacaccattttgctatagattttttgaccactcaggtaattcttttctttgctcttcttgtttattattgagaaaatacttctgctctagcatcaatttggtccaaaatgaagggttgttgctataatctaattagtcttggcattattcttttgcttatgttgtttgtgcagttgaactgtttttccatgtaaacatttgctaatgttaatttgtatgccaaatgcaggatcgttctgacataatatgtcatggcgttgatgctataaacacggaaacgcaggaagtaagtacagttgctttcactcatgttgacctccatgtattgaacatttcctcacaatgacataaattgatttcttaggcttctgcgctcttactgtgagtttgtaggttataagattcatttcaaaagtgactttgctggcatcaggtggagctgggcatatctatccaagtactactaatccaccggtatgagtttcaatatcttttcctccataatattttcatttatgagggatgtcactccttataatcaataagataatcagagtcctaaacagtgatatggggggagaaggtgggaagggaatggtggctaatactgtaatagttaatttcatgactagcatacatttgcatcttattgttggcgataagcttcgtcacaaagtatctttcgtaactcataaggaccttaacaattgacattggtgcaaacaacattccctagagtatgaaacatggcctgattttaattatttaaaccctacagcacttgcatgttaagctaatgtgcaattagaaataagggctggctgccctaagccacaaaaagaggaaaaacccaaatatacccctgtacttcgtgaaaaggtctaagatttattctccctttgaagtttggctcgctggtgccctcgccgctaaacttttggactatatttacccctatttgctaacggaccttggtttgagacttaacaacaacaacaatatacccggtgtaatcccacaagtggagtctgaggaagcgtgtcaagataatagaaggaaaaagatatttaggagagaaacaataaattgcacaagacaagacaagatttaggtggttcgacaatttttgcctactccacggccacacaaagaatagctctttattaattgaagagagaaagaagaagttttgggatgatctacaaatgaaaatgtagacccctatttataagcatttgaatgccctgccgaggtaagcgcttacatcataagaatgtcgatgtaagcgcttacatcataagaatgctgaggtaagcgcttacatcacaagaatgtcgatgtaagcgcttacatcatattttcatctcttttcgatttttctttcttttgttttgtctactttcacatacaacaacaggtttggtcctatcaatctccctctcaaacctatgttacatcaagaaagaaaataaagaaagatttgctattctctggtggcgccttcactctatcagtcttgaaggctaactgaggcagtgcacagcctcagtttgtcaacaccgacaactttggtcaacatgtctgacgggttctttaatcctggtatcttttgtagggaaagagttccttcatttatcaactctcggatatgatgatacctcaactggatatgcttcgttcttgcatgaaacactggattcttgtcaagatgaattgcactctggctatcgctgaaaagctcataattgtcctgttctttacctagctctttaagaaaattcttgagccaaatcatctcttttccagcttctgagattgccatgtactctgcttcagtggtagatagagcaacacttttctgaagtctggacatccaactaacagcagtaccaccaaaggtgaacatgtagcccgtggtactttttcgactatccagatcgccacctaaatttgcatcagtaaaaccttgtaagataatattgctctttttaaaacaaagtgccatacctgaagtgcctttgagatatcgcaatatccattttacaccttcccaatgctcctttcctggatctgacatgtatctactgacaactccaactgcatgggctatgtcaggtctagtgcaaaccatatcatacatcaaacttcctactgctgaagcatacagaactttggacatgtacttcctttcttcatctgtcttaggtgattggtcctttgacagatttagatgacttccaagtggagtgcttctggtctttgcatcatgaagactgaacctgcttagtaccttctgtatgtacttttcttgagacaactttaaggttccttccgacctgtttctgctaatcctcatcccaagcatttgcttagctggtcctaagtctttcatatcaaactcctccgccagttgttgcttaaccaagttgatctcatttatgctagatcctgcaattagcatatcatcaacgtacaacaataaaatgatataggattcatcaagatttttgatataacagcaatggtccatctcacatcgtgtgaaaccatttttatgcatgaatccatcaaatttcttgtaccattgtcggggagcttgtttcaaaccatacaaactcttcttcaacttacacacaaggttttctttaccagaaacttgaaaaccttcaggttgcttcatgtagatgtcttcttcaaggtcaccatgcaagaaagcagttttaacatctagctgctccaaatgcaaattttctgcagctacgatacttagcaccaacctgatagtagttaatttgactacaggagagaagatctcggtgtagtcaattccttccttctgctgaaagtcttttactactaatcgtgctttgtatctcttcttaccatcatgctcttccttgactctgtacacccacttgttctgcaatgccttctttccttttggtaactccgtaagtatccatgttttattcttttgaagagaattcatctcttctttcatggctagcttccacttatcagagtctatcacctgcattgcttcaacaaaatgctctggttctccagcatcagtaagaagtaaatagtgaagagagagttaatttatttggagcattcgtgactcttttagatctcctcaatgtaggttcatgagtaacagaatccgaatttgattcaggtcctgattccagatttggttctggatttgattctgtctctggttccacttcaggttcggcttctagttcttcttcaaattcggcttctagttcttcatcttcaatttcagaatcagttgtaatccctctagctacttcattttctgagatttcttctaactcaactgtttcagacattgtctgtttgctggtgttggttggttctacttcaagcttgtccttgtacatcacattttcattaaatgtgacattcctgtgtcttaggatctttctattcggatcatcccaaaaccgataaccaaaattatcatcaccatagccaataaagaaacatttctttgctttaggatcaagcttatctctatcattagagtttacatgcacataagcaacacaaccaaaaattttcagatgtgagagagttacctcctttcctgtccatacctcctcaggaatttcaaaattcagcggtacagagggtcccctgtttatgaggtaagctgccgtgttaacagcctcagcccaaaaatacttcggcaatccagaatgtattctcatacttctggctcgttcattcagggttctgttcatcctctcagcaacaccattttgttccggtgttccaggaactgtcttgatcattctgatcccattctccgagcaaaatgctttgaactcttggctatcatactctcctccattgtcagacttcagacattttaactttagacttgtctgattttcaacttcagctttccatcttttaaaggtaacaaatacatcagatttatttttcagaaaataaactcatacctttcttgtggaatcatcaatgaaggtgacataatagcgtgagcctcctagagaggttacaggagctggtccccacacatctgtatgcactagttccagcttctctttctttggcgtccttcccacctttgagaaactaactctcttttgtttcccgtaaatgcaatcttcgcacaaacctaattcaacatgttttaggtttgacaacttctttttggatgccaaaagcttcattcccttctcactcatatgcccgagcctccggtgccacaatgttgtatcacgaccatgatcaactgttgctatagtatctctttctattacagttgcatgcagtgttccccttttgaagcctcgtgccacaaccaaattccctttggttatcttccacgatccgttgtcgaatgttgttgtatatccttcatcgtcaatctgacccatagatatcagatttttcttgaggccaggaacatgtcgtacattttgcaatttccatagcgtgccttgtgaagtctttatataaacttcaccttttccggcaatgtcgagaggttcgccgtctgctagataaactttcccaaattttccagcaatataattatgcaataattctttgcatgatgtagagtgaaaggacgcacctgagtccagaatccaagattcaactggactgtctgcacaacaaattagtgcatcaccgacttgttcagcaattacatttgctgaattttcttccttcttcttctttggttctctacattgactactgtagtgaccctttttatcgcaattccaacaagtaatgtccttgcgatttttggattgtcctcttctccttgactttgatctgccacgaccataaatctgtcctctttggttgattctccccctgctttcggtactaaaagcagatcctggggaatcacttgattcttttcggcgaatatcttcgcttagaaccaagtctctaatatcattcaatttgagtttggtacttcctgatgaactgctaactgcagttactgttgcagaccaactctccggtagagatgatagtagaatcaacgccctgatttcgtcatcaattgttatattaacagaactcaactgagttaatattgtattaaactcattgatatgttccgtgactgatccaccttctgtcatttttaagtggaacaatcgacgcatcaaatacactttatttgaagcagatggcttctcatacatatttgataacgccttcatcaggcctgcagtggtcttctcgttaatgatgttaaacgccacatttcgtgttagcgtcaaacgaatcacaccaagagcttgacgatctaatagatcccaatccgctttggacatagtctccggtttcacctcggtcagaggtaagtgtaattttttctggtacaaataatcctctatttgcattttccagaatccaaaatctttgccattgaacttgtcaatcttaaccttcccttcttccgatgccatttttcacaaaaataatttatgtgaatagtgcttgtgaatagtaacgatgatcaatagtgtcgcactattcttgtgaatagtacctgcaccaatactgtacttttctaccaggattacactgtctgtgctctgataccaattgttgaggaagcgtgtcaagataatagaaggaaaaagatatttaggagagaaacaataaattgcacaagacaacacaagatttacgtggttcggcaatttttgcctactccacggccacacaaagaatagctctttattaattgaagagagaaagaagaagttttgggatgatctacaaatgaaaatgtagacccctatttataagcatttgaatgccctgctgaggtaagcgcttacatcataagaatgctgatgtaagcgcttacatcataagaatgctgatgtaagcgcttacatcataagaatgctgaggtaagcgcttacatcataagaatgctgacgcttacatcatattttcatctctttttgatttttctttcttttgttttgtctactttcacatacaacaacaagtgtaatacccgggtatattgttgttgttgttgttactcatactgctgctactcatctacgtgatcgagaagtcacaacaacaaattctgggcagaaccaaattggtacaaccatcccagatatttcagaggaggaaagaagactcttggatgcaatggtgagttctaatcccttaaatcctgtaaatcctacttgcttctagcactggaatgttgagtatgagcaggaacaaattgcaaaaaatagaacaacatcaaagcaaggcaatggtgacaaatacacttggtcaatctgcattgaagacaattgttatcgaccaaaatgttccacaacctgtgcacctggggagagacttgtatgaagacggagaggaagaagcaatgttacatcagtgtagagcagaggcagcaagaaaaggggatctatcaccaatgcatagcggcaaaggtaagagactcatacaaggaaatttagttgggacgacaaagttagtgattttttaaatgttaggcgacctccaatgagagttgccaaacaaaagaaggccgccccaactacatctacaaagtccaatcattcaaaaaagaaatcatgaattttgaatacatcttgaagaattggattgtgatgaaaaagagttacaaactgaagaaattacaagttcggacaagaagggacaatattttttcggaacaagtcggtgaaggttctattacggccgatagaggggtggcggctcgttgatggggttgtaaagttgtaatggtggtgaccggtgaaggttctattttggtgagaccatggaattgagagggggaaggtgctagctgagaaagtgttgaagtagtgaagcggtgagggagtctctgtggggagctgttggtgggttggtgaggttgtttggcggtttcagatgcagaggtgtaacaagtcggacaagaattggtcagacagggcagtttttctggcaattttttttttttaaattttttttgaaggttctgtggtgctcaaacttctatgaaattttcagggatggttaattatggttggggtggttgctgcctagaggattagataaaggtggaagtggttgtttagttatagagggagtactttgggcgacggtggagaatggtttggggtgagactttgggcagcaattgtttgcgaattggatggtgaaggttgactagatgaagtgggttttgggcaacaacatgttggggaatggaagcattactgtgttacaatggagaaggggaatagatggagatctttgcgggaaatgggggaaaatggcctaagggcagcgacggggtgcaggggttaatgggagagggttaaagggggagggaggtttattaattagccacgtgtgggacatgtcacatgtggcacattctggtgctaaactgagtttttgagattaactaaaaaagagatcaaatgatttttaatcatcagctgttagcaataagggtagatatagtccaaaagtttaagggcaccagtgagccaaactttaaaccaagggtaaatctagaccttttcacaaagtacaaggacaaatatggaccttccctcctacccctcccccccaaaaaaaaaaaaaaaaaaagaaacaataaagattctgggtattaacagatgatcctttccttggaagtgtggattcttatctcataagagatgaaggtaataaattcttattctatacaccaatatttttctgtacaataaaagcaagacacattgttcaaagttgtataacctgggttaggcatctactgtggcgctgttatgctcgttatcaattgtttttctcttacggtcatttctataagtttttggagctactaattggtggtggggcccgattctttttttatatttgaccatttgtgcctttatcaaggaacagaaaagttttaatttgttgaatgtgggcatgctggctgtaggttgcaactggagatggaatggctatggctcatcgagctcaagctgtaatttccaacatggagtaagtgatcctcagttgcattgcattcttattgtccaatatcactgtgtctgctttagtgagttgtgctgtaaaatctgctaatctagatttcatccattttttgctttcttgatttctgcatcctgttctgcaattcattctgaatttgcacttttgactaaaaatacaaggtatgttcaaaatgttgtgcggggtgacattggatctgacctgaatttttcaggataaagggcatcaaattttcttcattgaggggatttaattgatatagaaaagatttctcgactagcagtccgctctctaattgatggtcctcctttgatcgtcttttggatggtagacaagtctttgtttgcgaggttgatgaactatccccaacggttgcattattaattacaattctcttcttcatgttgccaggtttgtgcaattccatccaactgccttggctgatgaaggccttcccaacagaccaagtgccagagagaatgcttttttgataactgaagctgtcagaggtgatggaggcatcctttacaacttagatatggagagatttatgccaatgtatgacaaaagagcagagcttgccccgagagatgtggtagcaagaagtatagatgaccagctcaaaaagcgtggcgaaaagtatgttcttcttgatatcagtcacaagcccagagagaaggttctgtctcattttcctaatatagctgctgagtgtctccgccatgggttagacataacacagcagccgattccggtggttcctgctgctcactacatgtgtggtggagttcgtgctggacttgagggtgagactaatgtgcaaggcctttatgtggcaggtgaagttgcatgtactggtttacatggtgctaaccgacttgctagcaactcgttgcttgaagcactagtgtttgcacgaagagctgtacaaccttcaattgatcacgtgaatgtgtctagaattgatcactgtgcttcaagttggtggccgcgacctgtagccccagtggtaataggagatacagtacttaacaaagtcattcgtcggacaagggaagtgaggaaagaactacagtcaatcatgtgggaatatgttggaattgttaggtctacctcaagactaaccgcagctgagaagagaatcaatgagttggagttggaatgggaaacatacctatttcagcatggctgggaaccaacaatggttggactagaggcttgtgagatgaggaatctcttctgttgtgccaacctggtagttagcagtgctctttctcgacacgagagtcgcgggcttcattacaccattgattttcctcatgttgtggaaagcaagaggttgccaacaatcatttttccttcacagcgaaatagctcgtggagctcacggcaattacacaggcagcagatatgttagatgctcttacctatttgccaatccttcctgctaaaacttgtcaagcgcagggcatgattagtttttaggtaaagaagatgcttatgggttattgtcattcttcctgccattacttttggggcagggcaacgtcattctttggtgaaaaaaatatatatctatacatacaacccatataattttgaatgtgtttccctattttattcttatatagcatattttattatctgctaacttcaagcctgtctagtactcacacgtcccaaaagaacaacaggttttaaagtaaaaagttaaaccatttaattttctgtctccatatagacatcaattttttgaatctttttaaataaaattaagggagatttgcacatatacacagtccaacacactgtattgcacctatgtaactaagtttttcacttttcacctgcatagccaacatttgttttgcaacaatgtatatacatctttaaacattattgtatatttgttgtaaacaatgtattaaccttgtataaaatgtataatagtaaggtgtttatacatacttacactgttatataaattatacagtgttatacaaaaattgagtgtttgattcaccttagaagcagttttagctggcaaagatcccccccccccagtctttgcactctcatccttgcttatattctgcactaattttctagttgttcccttgatttctttgtttgggatggagaaaggtgtgtggagggagttggttcgatgacttccgtttgagtttcttcttgtttcttggtatgatcagacttggttttggtagatgacctggtactagacttgggtttaagggtggtttggctagatttgatcatggtgaattttctaggtttaaaaattttcttagagccttacaggggagaagtagggatggcaatggggaaggccgggcgggttaagtcttcacctactaaatttttgccttgccttgcctcgtttagttctttgccccatttagatcatgccatgccctgccccgtttagccctaaacttaatagttctttcatttttatccatctaactagcgcaattgtttctaataatatttagtaaatggtctcctacttcatcgattctgtaggagcctaaattgtctaaaaaaaaaacgccatcttccttcgtgcagtttggtatcttataccaatcgagagagataatgttttttccgtactttgtaaacgaactacaagtcaacattatgttgaacatttcgtactctgtaaacgaactacaagtcaacattatgtagtacaagtcaacattatgtattcgacgggaagcgtcacagcctaggttaggaacacccccgagaaaccttacaataggcagatcacctcttttattatagtagatagacaacatttgtggactacgataaatgttttcaaccaatctgacattgtaaatgcacatgtaatgccatgtatcagttcatacatgtggtaatttaatgaaggattggaaatatacatttttattttacaatagaagaatgctttattagttctttgtgcttgccaatctgaaagaaatcatttgatattctgtgacatcatgaagtcaacaccaaaaaaagtttaaatggttgatagattctttttgtcagttttcacacaggtaacatctgctgcaaatagaaagtcctcttctctgccaattatcttggctaagacatgctgcctcgacagcattccccacaaagcagggaattttggtgtgttgtttttgtcctccgtgttatcttttactatccagcttttggagaagattgtagcaactttggacaccctatacagtacctatatcataatcagaactactggtctataaactccattactttttcactttgttccgcaatcacctttgaggttgttgtatagagcaagattgaggttgtcgtaaatgtatatttatcaccatgactgttttcatggtaaatgtcctgattaaggtggcaagaccataatgcatgtgttgaatttaccatctgcacatatgaatggagaagaaaaaatgttaaaacaaaaaaagaacaaaaaaagacaatggtaataaagacgatgaactaagttcaaagcggctgcaaaagtgtgaaaggtgactgttctctatcattaaagtttatcttaaactattgatgtcattcagggttgacaaaacagtcaccaaatataagcatttttgttcggggttgaactacagagagtaggaattcatccttcaatgtccctgtttcaatccaactatgtgtgcaaaattttatcttccttttaatccccatattcaacatgatactgctgtatcacgttgtttagctgcactgctaaaacataaaattgtagggagcatgtaaattttacatagcacatccttccatagatgtaacaggaggtgtatataaaagaatgtataatttgccatcaatcagaagtaaaggttatgcactaaccattcatagaaagtgatataatcgatgtacttgatgcaaaattttaaggtgctcttcaaattatcacggcaaaaaggcaggaccctgatcttgtattcctgcgaggttgagaaaaggaaaaccgttctcagtcaggttcccaaaatagtgaaagagatgaatacagagaatgtaggtatgattcttacttctcaagaaaacataggtacatttaccaaattgtaacggcaaaaagatttatgtgaaaggttttagccttgactatgaagaagtcgcatttgagatgagaaagtatcgccagctatggtgaattatagtaactaaaggtgccttgcatcacatatcatgtcaatatgtagatagtttatatgtaaatagataactctcatgtcttttttttttgcaagcacatatcatccctgaattgaggggattgagcttgctgtcaaagcataaactcctggaaaagctaaatgaagtctctgatttgtagtgcagagta

SEQ ID NO: 69 - DNA, 23389 bp, Nicotiana tabacum
  misc_feature (18379)..(18541): n is a, c, g, or t
gcttccttggccaacaatcagttaatttgtaacttcgaattcgagttcaattctacttcggagcgccatttttgccccgttaaggtaactgtattgttcaaaactttttttgttttgtcgatctatttttttttgttttgttttggaataataactatagttgtaattttttgggtgggggatgtggttgtaatttagtctagggttctgttaggttggggatgctagaatcttgagaagctttataaatatacgaacatgcagttgtatgataaactgatagccggtagatcctgttgttgcgaacatgctatgctagctcaattctgctctctgttccctttttctactgttttctttccctggtaaagcaacacaggctgacacaatcctagcccaaatgagagtaacaaagtttccagtctttagaaggtgaaatctataagcaaatagatgtgaatgtaagtgccttctggggcatacgattaacaaatagacgtgaatttaaatcactgcaggaattgagagaagaaatatagagtgtgttcggtataactgaaaatgttttcacttattctccagtatttggctggtgagggcaaaatatttccggagaatatttacaaatgtttgtttggtgagtggaaattgtttcctaatgttgttacaaaataatttactttttgatttcatttaggccccttaaagttcttgaaagattaactgcagaaaaaagtattcaacatgacatgtcattcttgtaagaacaagtcattaagaaaaagaaaaataatatattaaaattagaaagtttctaaatatatgaaaatgtcaatcttttgtaaataattcaagaaaatgaataatgacagtaatttaaaagtatcacagatttacataaagaaaggaaaaggaaaagagagaatggtacatgaaattttaaatgctttggctagattcaaattccatactcctattaaaagaaatgcctgacaggtaagaacatataggtactgttgtgtcaacatgcaatagcatttggtcactttggagagagtatagagaaaaagagaaaatggcagagggaagtgggagggaggcaagagccgattgtctagcgccaaaaagtttgatatgttctggatattggaaattgactttccttgggttcttaggtaagttagtttcatcaaaattaaaggaaaatgttttctttaggaaaatgtttccccaacaatttaggccaaccaaacatggtaaaattggaaaagattatcaagaaaatgttttctttcataccaaatacacccataagtaggagggattgtgataaattttgcaagttgtttatgtattttcagagatctatttacctgtcatacatgttctacaaaacacgagtccatgtatatatcattgcacttctcctttacaacttatttaatttctatttaaacagctttagcgcgtaagagctgttcatttccttgaacaccattgccaaagaacggtttaatgagggaaaatgaaaatttagctatgttggcaagtcctgagtcttagagcaaatgatcttcattgggtcttattgtttccttgcaatacttgttcagtcttgtaagttctgattttcgctaaaacaactctttttagtcgtcacttgttacttacaatttcctttctcctaatagaaacgtgtccggaaagctgacttttggccctgtatgtgtttctggtttttggagccttcagaatgatagtactagctgttcaggtgtctattgagggtcttcatcaaagcaacagtaaggaaatagttagaaaaactgaaaaggacttctccttaacgtgtttcagtctcttgattttaaaggaaatgcattttgtagatacattggcattcattgaaaatggccttgactcaatacctatgtcatgtgacatcaggaagggaaagcaatgatttctctttctgtttcagtaataagtgatgaagtcttgtggcaacttccatttgtaaattcattttgtacaagtggattatagaaaattagttgataagttcatacctttcttttctctactttttctcttgcaatatgagatatcacaggttagagacatgatgcacattcatttgtggttcacttgaatgagaaaaaagtatatgtttcttctttttatgtttcgtttccttttggttttcagtatctggtatcgaagttgtgtaataaacagtttgttccacgcatgtgctgctgcagcattaacatggactagccatcttgtcgtaggagttcaatttgtggaattccggtttaagcccatcaactgtggaatctctaaatattttcattgaattcaccatacgttagatgatatgttttctcatggtcctttcaagcacttctccttctgtttaaatgtctccacatgcttttctgccccttcaatatcagaatttgtctaaaagttcctttttctttaataaatctactgctccaaatgaatgatagaagagttgtaaagagttctgacttcaagaccaagcacagttttggttgggctttcaaattagcttataggaagttgttcctaagatcgtcctgaaacaaaatcttttctttttgtagcttctactgtattcattcatgctttaatgcaatttataacaaggtttcccctaaatatccagagtctttaattttgctttcgagtcccagctgcgcaaaacgtattaccgaagaatagttttctgggagatgttacaagagtttggttagaagggtctttcccttctaaagtgtttggttcaagttatctaaatgtcaagagccaatattttgttattaagctcaattccttgccctgtttgggtgtttttagaggtaatcaagatgatttttaaatgtttagtttcactaacattctaacctcagaattgggtgtgccaatctgatatcaattcctttgacttggattgtcagtcaggaagatcatatggcaactggtatcgcttcaggaagcggacagttacatttgaggaagcctgtctactggaggagtagctatggaaaagctcactgtcattccaatgcgatcctgaatggcatgcaaaaccagatcccttggtccgtattaggatgatgtttcttcgcctatctctcctctctatctttccctgctttattatcttcattctattgccccttctcctctcttttgggggaataattgtcaaaatgttttattttggagctttcaagatgttattacattccaatttgtacggacataggcattcacgtgttggctgttggactgtttattcctcccatgagaacttactggaaagaatctttgtatacgtgtttaggcataaaccagtaatatcttttttcatgagataccagaatcctaaaagttttttttttgagtcatttcctgattctttaggaaaaaaagaaaggttatcattttcattttctggtggtgatatgctacttaaattttccaggtcttattgggtttccaaattcttgcgagttcatagaagtaactactcacaatgtcaagtgaaaacaaactggaagtctcacaccggaacaatcaattcttgccagagagatggctcaactaggtattttgattttgctgtgattggtagtggaattgctggccttagatatgctctagaagttgcaaagcatggaactgtagctgtgataaccaaggctgagcctcatgagagtaacactaactatgctcaaggtggtgtaagtgctgtgttctgccctatggattcagtggagagccacatgcaagacacaattgtggcaggtgcttacctctgtgatgaggagactgttagagtaagttcacagaatattattgtctcttcagttccgtgaagcagtttgccctttttcagttttttctctttggaagctgtttcctttgcttttccaaatttttccaggactgcttggttggatgaataggaaagttctccatctttcaggttgaaacgaaaggaactttctgtttagacggcttttgccacaggatctagaactgccaaaaaatggaaaagggtaagagcaatcgggcagttaggcttgttttcaattagaagctgaagagccaagcaataatactaaagaaaggctctatgcctattccttccttctgatgtaagtgcttacaagttggaaccgaagaaagagttggagagttgagaaaccaatggttggtaatatggacgacttcctctggtttatgtagtgctcctattcttcatggttcagattgttgaatttgtctttgaacatcgtgagaaggcacgggagaaaatatgattgatattattctcatatgttaaacatgatacaatgagccctgtatatacataacatgtcctactcctaatacatatgggattagggttacataactattctaacactcccctcaagctggtgcatataaatcatatgtaccgagcttgttacatatgtagttaatacgaggaccagtgagagacttggtgaaaatatctgcaagctgatcattcgacttcacaaactttgtagcaatatctcccgagagtatcttttctctgacaaaatgacagtcaatctcaatgtgtttagttctctcatgaaacactggatttgatgcaatatgaagagcagcttgattatcacacacaagtcccatctgactaatctcaccaaatttcaactccttgagcaactgtttgatccaaattagctcacatgtcaccatagccattgctcgatattctgcttttgcactagaccgagcaaccacattctgtttcttgctcttccaagataccaaatttcctcctactaagacacaatatccagaaatagaacgtctatcagaaggtgatcctgcccaatcagcatctgagtatccaacgatctgctcatggcctcgatcctcaaacaataaacctttgcctggagctgattttatataccgaagaatacgaacaactgcatcccaatgactatcacacggagaatccataaactgactcacaacactcacaggaaaggaaatgtcaggtcttgtcactgtaaggtaatttaatttaccaaccaaccgcctatatattgtaggattgctaagaggctccccctgtcctggcagaagtttagaattcggatccatcggagtgtcaacaggtctacaacctgtcattcctgtctcctcaagaatatctaaggcatacttccgttgtgagatcacaatatctgagctagactgagcgatctcaatacctagaaaatactttagtttgcccagttccttagtctgaaagcgttgaaagagatgttgcttcaatttagtaataccatcctggtcattgccggtaataacaatattgtcaacatagaccaccggataaatatagagactcgaagcaaaatgccgatagaatacagagtgatcagcttcactccgagtcatgccaaattcctggataactatgctgaacttaccaaatcaggctcgaggagattgctttagaccataaagtaatcggcgcaagtgacatactaggccacgagactccccctgagcaacaaacctaggtggttgctccatataaacttcatcctcaaggtcaccgtgtaaaaaaacattcttaatgtccagctgatagagtggccaatggcgaacaacaaccatggatagaaaaaggcggactgatgctatcttagccacgggagagaaggtatcactgtaatcaagcccaaatatctgagtatatcccttggcaacaagacgagccttaagacgatcaaccttaccatccggatcaaccttgactgcatacacccaacgacaaccaacactagatttacctgaaggaagagggacaagctcccaagtaccactcgtatgtaaatcagacatctcgtcaatcctgtcgccatcctggatgagacaatgcttcacctgtagacttagggatggaaacagaggacaaagaagatagaaaagcataatagggtgaagacaaacgatgataacttaaaccgacataatggggattaggattaagggtggtccgtatacctttccgaagtgcaatcgatgtactaggaagagacaagtccgcagtaggaccagggtcaggtgcaggacgtgaatcagctgggcctgatgctgggtgcagatgacgatggtatgtcaagagtggtgttcctgtggcagggagtgtaagaggagccacactagactccccaacggttggaatgggtaagacttctgtggcggaaggtgaagaaggagatatagtagaatccttaaaggtcggtataggtaagacctcagatatatcaaggtggtcagaagaggtaaagaaaggtttagactcaaaaaatgtgacgtcggaggacataaagtacctacgaagatcaagtgaataacaacgatatcccttctgaacacgagaataaccaaggaagacacacttgagagcacgaggagctaacttatctttcccaggggctaagttatgaacgaaacaagtgctcccaaaaacacgagggggaacagagtataagggtgacgggggaaacaatactgcatacaaaatctgattctggatgggagatgaaggcatccaattaaccaaataacaagctgtgagaactgcatcgccccaaaaacgcaacggaacatgagattcaatgagaagtgtgtgagcagtctcaatgatgtgcctattctttctatctgcaaccctattttgctgaggggtataaggacaagaggtctgatgaataatttcttgagaagtcataaactggtaaaattgagaggataaatactctaaggcattatcactgcgaaaagtgcgaataaaaacacgaaattgatttttaatttcagcacaaaaattctggaatatagaaaacaactcagaacgatctttcattaagaaaatccaagtacatcttgaatgatcatcaataaaactaacaaaataacgaaatcccaaggttgaattgactctactaggaccccatatatcagaatgaactaaagaaaaaatagactctgcatgactctcaatactacggggaaaggaggctcaggtatgtttctcgagctgacatgactctcattctaatgtagataaactagacaaactaggcaccatcttctgaagcttggataaacttggatgtcctaaatgtctgcgaattaggtctggaggatctgtaactagacatgccttggaggaattgagtgagttaaggtagtaaaggccttctgattcaagtcttgttccaatcgtctgtcccgtactgcggtcctgcataataaaagaatcatcaataaaatatataccccaatggagggcacgagtcaaatgactaacagatgtaagattaaaaggacagccagggacataaagaacggaatctagagtgacagagggtaggggattcgcttgtccaacaccttttactttagtttgagacccattggctaaagtaacagtgggaagagactgtgaatacgcaatatttgacaaaagtgatttattaccaaaaatatgatcagaagcggctgagtccacaatccattgtccaagagtactagactgggaaacacaagcaaaagaattaccagcaacagaagtatcagtctgagcaatagaggctacttgtggagatgtttgcttatttgctcgatattgaaggaactcattatactccccttcagataaagaaaatccctggttacctgtagtctcggtctgagcaacataagcatttttgggtgggcgaccatgtaaagaatagcacacgttactagtgtgtccaagtttatgacaataagagcacttgagtctagatttccaaaacgacctcctcctcgtctattctccatagtttgagatgcccgattgtccactgactgggatacgaggacagatgagtcaagtgtctgtgatgagctcactgggtgacttggtgctgcagcaaggcgaagtaatcgagagaataattcatcaactgtggggacagtcggtctagccaaaatctggtcacgtactgaatcaaggtcattagggagtccagcgagtgtaagaactacaatatcctctgtcgttgctcttgttgcttttcaatactagcagaaactggcatcaacgtctcaaattcttccatgactgcctgtacttgttccaagtaagtagatatatccaattcctgtttcttcaagcttgtcattcgcaatattacatcatagagacgagatatgtcattagtgtataaattacgagccttttcccaaactaaataacatgtatggaatggacggaacaagagcatcaatttggaatcaatagatcgccacaagatactacataactgagcattgaccttctcccaaagtgttttggccttttcatcaccttcgctagccttttttgttaaatgatcttgaactcgttgacctttacaccacaactcgaaagacgaagcccaagctaagtagtttgaacctcccattaaaggttctgaggtaatcgtaacaccggaattgccagaacccgggtttttagacccgaaagcatcgactcccaaagacatcgttggattatcaccaaataacagaaagaatcaactgacaacttgctgaaacaggtgaaggaaacactgtttttgccggaaaattactgtagctgccggaaaaagtcggtgtagtcgccggaaaaactcaaagtggtcggaatcaaacgaaaaaggtatggagactcggaattactaggcgatccgactgtccaactggaagtttttcaaaaaaatggttggaacagtgctcacgcgccagtgcgtggggcgcttgggtcagatctcgccagaaagtttttggcgcgtgagggcgcgtgtacgtgagttttccggtggggtttactagggtttggtcgccggagcctgaggagtcttgtggtgttattggttttttgcacacaccaacaaaaattgatgtgattacgagcagccttctaagtcgccgtaaaattgcacggcgacgaggtctttcttcccggaagtcgctggaatgatgcacaacgataggtttctcactaaagctctgataccatgtgagaaggcacgggagaaaatatgattgatattaaacatgatacaatgagccctatatatacataatatgtcctactcctaatacatatgagattaggattacataactattctaacaaacattatgaaaagagagtgaaggtgacatgcaggaaggaagagataaggataagacaggaaattcacatgtgttgtcttttggttttattttgggatttcatttagtttgtgccacagtaccatgtttttttttcttaatgagaacacacttctgacttccctaaatcagcaccaattttctgagggtaactgctgataaggatagacactccaaggttatccaggattcctagcttaagttgtatcatataagtttctctcctatcccctcaagagtcctatgtacagaaaactctatcccttctctctcgagctttagctccggagtccatttacttttgttaatgctaacaactcttgcggagttgtgaagtgccttcttctgccgagagtagtaaggcccaatggacttcgcatctagtaggcccattatcaacatacaatgagggagaagggatagagttctctgtatataactcttgtggggataagagagaatcttatatgatacaacttaagctaggtgttagcggaaacgtaaaagaaagaacacaagatttaacgtggttcggatcaaaataatcctacgtccaccagagaacaattgcccttttaatattaacaaaggaaggggagatttcccaattacacttaagagaatttctctcttaactctctactcactacaatgtattgtattattttgggatgatttctacaagtgaaggagtgcatctatttatataggtaaagatgacatcaagaggaggtagtttgatgtcatgggtgacatcaaaggaggaagcttcctcctagcatccacaccaactctttccaccaactcttccaattggcatgccattgttgactaaacataaaccaacattttcagcatgccattgttaactaaacataaaccaacattttcactagggatcctggattgccttggagtgtctatccttatcaaccgcttagtttgctgtatactattttcatttgtctctgtaaatatatactggtttcaaggaagttttgtgttgtgcttggtagatgggatatcacaactaatatcttcttatcagttgataaaatcctggtccatgtaattctgctttttatgcaatctatgttctaaatgaaatttatgagatggctgatttattactccaaaattgtgtttagtctactcttttaaaatcttcgtttttataagtatatctcctttctccaggttgtgtgtaccgaaggacctgagagaattagagaactgattgctatgggtgcttcattcgatcatggggaggacgggaatctgcatctagccagggaagggggccactcccatcgtcgaattgtccatgctgctgatatgactggcagagagatagaaagggccctattagaggcagtttttaagcatcctaatatacatgtgtttcaacaccattttgctatagattttttgaccactcaggtaattcttttctttgctcttcttgtttattattgagaaaatacttctgctctagcatcaatttggtccaaaatgaagggttgttgctataatctaattagtcttggcattattcttttgcttatgttgtttgtgcagttgaactgtttttccatgtaaacatttgctaatgttaatttgtatgccaaatgcaggatggttctgacataatatgtcatggcgttgatgctataaacacggaaacgcaggaagtaagtacagttgctttcactcatgttgacctccatgtattgaacatttcctcacaatgacataaattgatttcttaggcttctgcgctcttactgtgagtttgtaggttataagattcatttcaaaagtgactttgctggcatcaggtggagctgggcatatctatccaagtactactaatccaccggtatgagtttcaatatcttttcctccataatattttcatttatgagggatgtcactccttataatcaataagataatcagagtcctaaacagtgatatggggggagaaggtgggaagggaatggtggctaatactgtaatagttaatttcatgactagcatacatttgcatcttattgttggcgataagcttcgtcacaaagtatctttcgtaactcataaggaccttaacaattgacattggtgcaaacaacattccctagagtatgaaacatggcctgattttaattatttaaaccctacagcacttgcatgttaagctaatgtgcaattagaaataagggctggctgccctaagccacaaaaagaggaaaaacccaaatatacccctgtacttcgtgaaaaggtctaagatttattctccctttgaagtttggctcgctggtgccctcgccgctaaacttttggactatatttacccctatttgctaatggaccttggtttgagacttaacaacaacaacaatatacccggtgtaatcccacaagtggagtctgaggaagcgtgtcaagataatagaaggaaaaagatatttaggagagaaacaataaattgcacaagacaagacaagatttaggtggttcgacaatttttgcctactccacggccacacaaagaatagctctttattaattgaagagagaaagaagaagttttgggatgatctacaaatgaaaatgtagacccctatttataagcatttgaatgccctgccgaggtaagcgcttacatcataagaatgccgatgtaagcgcttacatcataagaatgctgaggtaagcgcttacatcacaagaatgtcgatgtaagcgcttacatcatattttcatctcttttcgatttttctttcttttgttttgtctactttcacatacaacaacaagtttggtcctatcaatctccctctcaaacctatgttacatcaagaaagaaaataaagaaagatttgctattctctggtggcgccttcactctatcagtcttgaaggctaactgaggcagtgcacagcctcagtttgtcaacaccgacaactttggtcaacatgtctgacgggttctttaatcctggtatcttttgtagggaaagagttccttcatttatcaactctcggatatgatgatacctcaactggatatgcttcgatcttgcatgaaacactggattcttgtcaagatgaattgcactctggctatcgctgaaaagctcataattgtcctgttctttacctagctctttaagaaaattcttgagccaaatcatctcttttccagcttctgagattgccatgtactctgcttcagtggtagatagagcaacacttttctgaagtctggacatccaactaacagcagtaccaccaaaggtgaacatgtagcccgtggtactttttcgactatccagatcgccacctaaatttgcatcagtaaaaccttgtaagataatattgctctttttaaaacaaagtgccatacctgaagtgcctttgagatatcgcaatatccattttacaccttcccaatgctcctttcctggatctgacatgtatctactgacaactccaactgcatgggctatgtcaggtctagtgcaaaccatatcatacatcaaacttcctactgctgaagcatacagaactttggacatgtacttcctttcttcatctgtcttaggtgattggtcctttgacagatttagatgacttccaagtggagtgcttctggtctttgcatcatgaagactgaacctgcttagtaccttctgtatgtacttttcttgagacaactttaaggttccttccgacctgtttctgctaatcctcatcccaagcatttgcttagctggtcctaagtctttcatatcaaactcctccgccagttgttgcttaaccaagttgatctcatttatgctagatcctgcaattagcatatcatcaacgtacaacaataaaatgatataggattcatcaagatttttgatataacagcaatggtccatctcacatcgtgtgaaaccatttttatgcatgaatccatcaaatttcttgtaccattgtcggggagcttgtttcaaaccatacaaactcttcttcaacttacacacaaggttttctttaccagaaacttgaaaaccttcaggttgcttcatgtagatgtcttcttcaaggtcaccatgcaagaaagcagttttaacatctagctgctccaaatgcaaattttctgcagctacgatacttagcaccaacctgatagtagttaatttgactacaggagagaagatctcggtgtagtcaattcattccttctgctgaaagtcttttactactaatcgtgctttgtatctcttcttaccatcatgctcttccttgactctgtacacccacttgttctgcaatgccttctttccttttggtaactccgtaagtatccatgttttattcttttgaagagaattcatctcttctttcatggctagcttccacttatcagagtctatcacctgcattgcttcaacaaaatgctctggttctccagcatcagtaagaagtaaatagtgaagagagagttaatttatttggagcattcgtgactcttttagatctcctcaatgtaggttcatgagtaacagaatccgaatttgattcaggtcctgattccagatttggttctggatttgattctgtctctggttccacttcaggttcggcttctagttcttcttcaaattcggcttctagttcttcatcttcaatttcagaatcagttgtaatccctctagctacttcattttctgagatttcttctaactcaactgtttcagacattgtctgtttgttggtgttggttggttctacttcaagcttgtccttgtacatcacattttcattaaatgtgacattcctgtgtcttaggatctttctattcggatcatcccaaaaccgataaccaaaattatcatcaccatagccaataaagaaacatttctttgctttaggatcaagcttatctctatcattagagtttacatgcacataagcaacacaaccaaaaattttcagatgtgagagagttacctcctttcctgtccatacctcctcaggaatttcaaaattcagcggtacagagggtcccctgtttatgaggtaagctgccgtgttaacagcctcagcccaaaaatacttcggcaatccagaatgtattctcatacttctggctcgttcattcagggttctgttcatcctctcagcaacaccattttgttccggtgttccaggaactgtcttgatcattctgatcccattctccgagcaaaatgctttgaactcttggctatcatactctcctccattgtcagacttcagacattttaactttagacttgtctgattttcaacttcagctttccatcttttaaaggtaacaaatacatcagatttatttttcagaaaataaactcatacctttcttgtggaatcatcaatgaaggtgacataatagcgtgagcctcctagagaggttacaggagctggtccccacacatctgtatgcactagttccagcttctctttctttggcgtccttcccacctttgagaaactaactctcttttgtttcccgtaaatgcaatcttcgcacaaacctaattcaacatgttttaggtttgacaacttctttttggatgccaaaagcttcattcccttctcactcatatgcccgagcctccggtgccacaatgttgtatcacgaccatgatcaactgttgctatagtatctctttctattgcagttgcatgcagtgttccccttttgaagcctcgtgccacaaccaaattccctttggttatcttccacgatccgttgtcgaatgttgttgtatatccttcatcgtcaatctgacccatagatatcagatttttcttgaggccaggaacatgtcgtacattttgcaatttccatagcgtgccttgtgaagtctttatataaacttcaccttttccggcaatgtcgagaggttcgccgtctgctagataaactttcccaaattttccagcaatataattatgcaataattctttgcatgatgtagagtgaaaggacgcacctgagtccagaatccaagattcaactggactgtctgcacaacaaattagtgcatcaaagacttgttcagcaattacatttgctgaattttcttccttcttcttctttggttctctacattgactactgtagtgaccctttttatcgcaattccaacaagtaatgtccttgcgatttttggattgtcctcttctccttgactttgatctgccacgaccataaatctgtcctctttggttgattctccccctgctttcggtactaaaagcagatcctggggaatcacttgattcttttcggcgaatatcttcgcttagaaccaagtctctaatatcattcaatttgagtttggtacttcctgatgaactgctaactgcagttactgttgcagaccaactctccggtagagatgatagtagaatcaacgccctgatttcgtcatcaattgttatattaacagaactcaactgagttaatattgtattaaactcattgatatgttccgtgactgatccaccttctgtcatttttaagtggaacaatcgacgcatcaaatacactttatttgaagcagatggcttctcatacatatttgataacgccttcatcaggcctgcagtggtcttctcgttaatgatgttaaacgccacatttcgtgttagcgtcaaacgaatcacaccaagagcttgacgatctaatagatcccaatccgctttggacatagtctccggtttcacctcggtcagaggtaagtgtaatttttctggtacaaatagtcctctatttgcattttccagaatccaaaatctttgccattgaacttgtcaatcttaaccttcccttcttccgatgccatttttcacaaaaataatttatgtgaatagtgcttgtgaatagtaacgatgatcaatagtgtcgcactattcttgtgaatagtacctgcaccaatactgtacttttctaccaggattacactgtctgtgctctgataccaattgttgaggaagcgtgtcaagataatagaaggaaaaagatatttaggagagaaacaataaattgcacaagacaacacaagatttacgtggttcggcaatttttgcctactccacggccacacaaagaatagctctttattaattgaagagagaaagaagaagttttgggatgatctacaaatgaaaatgtagacccctatttataagcatttgaatgccctgctgaggtaagcgcttacatcataagaatgctgatgtaagcgcttacatcataagaatgctgatgtaagcgcttacatcataagaatgctgaggtaagcgcttacatcataagaatgctgacgcttacatcatattttcatctctttttgatttttctttcttttgttttgtctactttcacatacaacaacaagtgtaatacccgggtatattgttgttgttgttgttactcatactgctgctactcatctacgtgatcgagaagtcacaacaacaaattctgggcagaaccaaattggtacaaccatcccagatatttcagaggaggaaagaagactcttggatgcaatggtgagttctaatcccttaaatcctgtaaatcctacttgcttctagcactggaatgttgagtatgagcaggaacaaattgcaaaaaatagaacaacatcaaagcaaggcaatggtgacaaatacacttggtcaatctgcattgaagacaattgttatcgaccaaaatgttccacaacctgtgcacctggggagagacttgtatgaagacggagaggaagaagcaatgttacatcagtgtagagcagaggcagcaagaaaaggggatctatcaccaatgcatagcggcaaaggtaagaggactcatacaaggaaatttagttgggacgacaaagttagtgattttttaaatgttaggcgacctccaatgagagttgccaaacaaaagaaggccgccccaactacatctacaaagtccaatcattcaaaaaagaaatcatgaattttgaatacatcttgaagaattggattgtgatgaaaaagagttacaaactgaagaaattacaagttcggacaagaagggacaacattttttcggaacaagtcggtgaaggttctattacggccgatagaggggtggcggctcgttgatggggttgtaaagttgtaatggtggtgaccggtgaaggttctattttggtgagaccatggaattgagagggggaaggtgctagctgagaaagtgttgaagtagtgaagcggtgagggagtctctgtggggagctgttggtgggttggtgaggttgtttggcggtttcagatgcagaggtgtaacaagtcggacaagaattggtcagacagggcagtttttctggcaatttttttttttaaaattttttttgaaggttctgtggtgctcaaacttctatgaaattttcagggatggttaattatggttggggtggttgctgcctagaggattagataaaggtggaagtggttgtttagttatagagggagtactttgggcgacggtggagaatggtttggggtgagactttgggcagcaattgtttgcgaattggatggtgaaggttgactagatgaagtgggttttgggcaacaacatgttggggaatggaagcattactgtgttacaatggagaaggggaatagatggagatctttgcgggaaatgggggaaaatggcctaagggcagcgacggggtgcaggggttaatgggagagggttaaagggggagggaggtttattaattagccacgtgtgggacatgtcacatgtggcacattctggtgctaaactgagtttttgagattaactaaaaaagagatcaaatgatttttaatcatcagctgttagcaataagggtagatatagtccaaaagtttaagggcaccagtgagccaaactttaaaccaagggtaaatctagaccttttcacaaagtacaaggacaaatatggaccttccctcctacccctccccccaaaaaaannnnnnnnnnnnnnnnnnnnnnnnnnnnnnnnnnnnnnnnnnnnnnnnnnnnnnnnnnnnnnnnnnnnnnnnnnnnnnnnnnnnnnnnnnnnnnnnnnnnnnnnnnnnnnnnnnnnnnnnnnnnnnnnnnnnnnnnnnnnnnnnnnnnnnnnnnnnnnnnnnnaaaaaaaaaaaaaagaaacaataaagattctgggtattaacagatgatcctttccttggaagtgtggattcttatctcataagagatgaaggtaataaattcttattctatacaccaatatttttctgtacaataaaagcaagacacattgttcaaagttgtataacctgggttaggcatctactgtggcgctgttatgctcgttatcaattgtttttctcttacggtcatttctataagtttttggagctactaattggtggtggggcccgattctttttttatatttgaccatttgtgcctttattaaggaacagaaaagttttaatttgttgaatgtgggcatgctggctgtaggttgcaactggagatggaatggctatggctcatcgagctcaagctgtaatttccaacatggagtaagtgatcctcagttgcattgcattcttattgtccaatatcactgtgtctgctttagtgagttgtgctgtaaaatctgctaatctagatttcatccattttttgctttcttgatttctgcatcctgttctgcaattcattctgaatttgcacttttgactaaaaatacaaggtatgttcaaaatgttgtgcggggtgacattggatctgacttgaatttttcaggataaagggcatcaaattttcttcattgaggggatttaattgatatagaaaagatttctcgactagcagtccgctctctaattgatggtcctcctttgatcgtcttttggatggtagacaagtctttgtttgcgaggttgatgaactatccccaacggttgcattattaattacaattctcttcttcatgttgccaggtttgtgcaattccatccaactgccttggctgatgaaggccttcccaacagaccaagtgccagagagaatgcttttttgataactgaagctgtcagaggtgatggaggcatcctttacaacttagatatggagagatttatgccaatgtatgacaaaagagcagagcttgccccgagagatgtggtagcaagaagtatagatgaccagctcaaaaagcgtggcgaaaagtatgttcttcttgatatcagtcacaagcccagagagaaggttctgtctcattttcctaatatagctgctgagtgtctccgccatgggttagacataacacagcagccgattccggtggttcctgctgctcactacatgtgtggtggagttcgtgctggacttgagggtgagactaatgtgcaaggcctttatgtggcaggtgaagttgcatgtactggtttacatggtgctaaccgacttgctagcaactcgttgcttgaagcactagtgtttgcacgaagagctgtacaaccttcaattgatcacgtgaatgtgtctagaattgatcactgtgcttcaagttggtggccgcgacctgtagccccagtggtaataggagatacagtacttaacaaagtcattcgtcggacaagggaagtgaggaaagaactacagtcaatcatgtgggaatatgttggaattgttaggtctacctcaagactaaccgcagctgagaagagaatcaatgagttggagttggaatgggaaacatacctatttcagcatggctgggaaccaacaatggttggactagaggcttgtgagatgaggaatctcttctgttgtgccaacctggtagttagcagtgctctttctcgacacgagagtcgcgggcttcattacaccattgattttcctcatgttgtggaaagcaagaggttgccaacaatcatttttccttcacagcgaaatagctcgtggagctcacggcaattacacaggcagcagatatgttagatgctcttacctatttgccaatccttcctgctaaaacttgtcaagcgcagggcatgattagtttttaggtaaagaagatgcttatgggttattgtcattcttcctgccattacttttggggcagggcaacgtcattctttggtgaaaaaaatatatatctatacatacaacccatataattttgaatgtgtttccctattttattcttatatagcatattttattatctgctaacttcaagcctgtctagtactcacacgtcccaaaagaacaacaggttttaaagtaaaaagttaaaccatttaattttctgtctccatatagacatcaattttttgaatctttttaaataaaattaagggagatttgcacatatacacagtccaacacactgtattgcacctatgtaactaagtttttcacttttcacctgcatagccaacatttgttttgcaacaatgtatatacatctttaaacattattgtatatttgttgtaaacaatgtattaaccttgtataaaatgtataatagtaaggtgtttatacatacttacactgttatataaattatacagtgttatacaaaaattgagtgtttgattcaccttagaagcagttttagctggcaaagatcccccccccagtctttgcactctcatccttgcttatattctgcactaattttctagttgttcccttgatttctttgtttgggatggagaaaggtgtgtggagggagttggttcgatgacttccgtttgagtttcttcttgtttcttggtatgatcagacttggttttggtagatgacctggtactagacttgggtttaagggtggtttggctagatttgatcatggtgaattttctaggtttaaaaattttcttagagccttacaggggagaagtagggatggcaatggggaaggccgggcgggttaagtcttcacctactaaatttttgccttgccttgcctcgtttagttctttgccccatttagatcatgccatgccctgccccgtttagccctaaacttaatagttctttcatttttatccatctaactagcgcaattgtttctaataatatttagtaaatggtctcctacttcatcgattctgtaggagcctaaattgtctaaaaaaaaaacgccatcttccttcgtgcagtttggtatcttataccaatcgagagagataatgttttttccgtactttgtaaacgaactacaagtcaacattatgttgaacatttcgtactctgtaaacgaactacaagtcaacattatgtagtacaagtcaacattatgtattcgacgggaagcgtcacagcctaggttaggaacacctccgagaaaccttacaataggcagatcacctcttttattatagtagatagacaacatttgtggactacgataaatgttttcaaccaatctgacattgtaaatgcacatgtaatgccatgtatcagttcatacatgtggtaatttaatgaaggattggaaatatacatttttattttacaatagaagaatgctttattagttctttgtgcttgccaatctgaaagaaatcatttgatattctgtgacatcatgaagtcaacaccaaaaaaagtttaaatggttgatagattctttttgtcagttttcacacaggtaacatctgctgcaaatagaaagtcctcttctctgccaattatcttggctaagacatgctgcctcgacagcattccccacaaagcagggaattttggtgtgttgtttttgtcctccgtgttatcttttactatccagcttttggagaagattgtagcaactttggacaccctatacagtacctatatcataatcagaactactggtctataaactccattactttttcactttgttccgcaatcacctttgaggttgttgtatagagcaagattgaggttgtcgtaaatgtatatttatcaccatgactgttttcatggtaaatgtcctgattaaggtggcaagaccataatgcatgtgttgaatttaccatctgcacatatgaatggagaagaaaaaatgttaaaacaaaaaaagaacaaaaaaagacaatggtaataaagacgatgaactaagttcaaagcggctgcaaaagtgtgaaaggtgactgttctctatcattaaagtttatcttaaactattgatgtcattcagggttgacaaaacagtcaccaaatataagcatttttgttcggggttgaactacagagagtaggaattcatccttcaatgtccctgtttcaatccaactatgtgtgcaaaattttatcttccttttaatccccatattcaacatgatactgctgtatcacgttgtttagctgcactgctaaaacataaaattgtagggagcatgtaaattttacatagcacatccttccatagatgtaacaggaggtgtatataaaagaatgtataatttgccatcaatcagaagtaaaggttatgcactaaccattcatagaaagtgatataatcgatgtacttgatgcaaaattttaaggtgctcttcaaattatcacggcaaaaaggcaggaccctgatcttgtattcctgcgaggttgagaaaaggaaaaccgttctcagtcaggttcccaaaatagtgaaagagatgaatacagagaatgtaggtatgattcttacttctcaagaaaacataggtacatttaccaaattgtaacggcaaaaagatttatgtgaaaggttttagccttgactatgaagaagtcgcatttgagatgagaaagtatcgccagctatggtgaattatagtaactaaaggtgccttgcatcacatatcatgtcaatatgtagatagtttatatgtaaatagataactctcatgtctttttttttttgcaagcacatatcatccctgaattgaggggattgagcttgctgtcaaagcataaactcctggaaaagctaaatgaagtctctgatttgtagtgcagagtat

SEQ ID NO: 70 - DNA, 28331 bp, Nicotiana tabacum
  misc_feature (15258)..(15427): n is a, c, g, or t
  misc_feature (23365)..(23555): n is a, c, g, or t
aacaaacccagtttaatcccatacgtggggtctggggagggtagtgtgtacgtagcgttacccctacctataaaggcagagaggcaaattgtttcctaatgttgttacaaaataattttctttttaatttcatttaagccccttaaagttcttgaaagattaactgcagaataaagtattcaacatgacatgtcattcgtgtaagaacaagtcactaagaaaaagcaaaataatatattaaaattagaaagtttctaaatatatgaaaatgtcaatcttttttaaataattcaagaaaatgaataatgacagtaatttaaaagtatcacagatttacataaagaaaggaaaaggaaaagagagaatggtacatgaaatttcaaatgctttggctagattcaaattccatactctattaaaagatatgcctaacaggtaagaacatataggtactgttgtgtcaacatgcatagcgtttaggtcactttggagagagtatagagaaaaagagaaaatggcagagggaagtgggagggggcaagaactgattgtctagtgccaaaacgtttgatatgttctggatattggaaattgactaaccttgggttcttaggtaagttagtttcaacaaaattaaaggaaaatgttttctttaggaaaatgtttcccccacaatttagggcaaccaaacatgggaaaattggaaaagattatcaaaaaaatgttttttcataccaaatacacccataagtaggagggattgtgatcaattttgcaagttgtttatgtattttcagagatctatttacctgtgatacatgttatacaaaacaagagtccatgtatatatcattgcacttctcctttacaacttatttcatttctattcaaacagctttagcgcgtaagagctgttcatttccttgaacaccactaccaccaacaacaacccagtaaaatcctactaatggggtctggggagggtggtgtgtacgcagaccttattcctatcccgaaggagtagagaggctgtttccgaaagaccctcggctcaagaaaacaaaaagacaaaaggacaaaaggagacaatattagtatcaccacagcaatcataggaaaaataagaacaccatgaaatccagaagaaagatgcaaagcaaaagcgatacctagtaaataggtcctgcactgaaaagcgaaatagtaagacacaacattgccactagctatcttagacaaaaatcctacctggctagtcccacaatggtacaaagtaaggcaagactcaactacctcctaacctacaaccctaatactcgacctccattgaacaccattgacaaagaaagatttaataagggaaaatgaaaatttagataggttggcaagtccttagtcttagagtaaatgatcttcattgggtcttattgtttccttgcaatacttgttcagccttgtaggttctgctttttgctaaaacaactctttttagtcgtcacttgtcacttacaatttcctttctcctaatagaaacgtgtccggaaagctgacttttggccctgtatgtgtttctgttttttggagccttcagaatgatagtactagctgttcaggtgtctattgaaggtcttcattgaagcaacagtaaggacatagttagaaaaactgttgctgaaacaaaaagagaaatcattgctttcgcttcctgatgttacatgacataagtattgagtcaaggccattttaaatgaatgccaatgtatctatgttcaggtgtctattgagggtcttcattgaagcaacagtaaggacatagttagaaaaactgaaaaggacttcttcttaacgtgtttcagtctcatgattttaaaggaaatgcattttgtagatacattggcattcatttaaaatggccttgactcaatacttacgtcatgtaacatcaggaagggaaagcaatgatttctctttttgtttcagcaataagtgatgaagtcttgtggcaacttccatttgtaaattcattctgtacaagtggattatagcaattagttgataagttcatacctttcttttctctactttttctcttgcaatatgagatatcacaggattagagacatgatgcacatacatttgtggttcacttgaatgaaaaaaaagtatacgtttcttctttttatgtttcatttccttttggtttttcagtatctggtatggaagttgtgtaatgaacagttttttacacgcatgttctgctgcagcattaacatggactagccatcttgtcgtgtgagtccaatttgtggaattccagtttaagcccatcaattgttgaatctctaaatattttcattgaattgaccatatgttagatgatatgttttctcattgtcctttcaagcatttctccttttgtttaaatgtctccacatgcttttctaccccttcaatttctgatattttctaaaagttcctttttctttaataaatctactgctccaaatgaatgaaagaagagttgtgaagagttctgacttcaagaccaagcacagttttggttgggctttcaattttagcttttaggaagttgttcctaagattgtcctgaaaccaaatcttttctttttgtagcttctactatattcgttcatgctttaatgcaattcataacaaggtttcccttaaatatccagagtctttaattttgctttcgagtcccagctgtgcaaaacgtattactgaagaatagttttctgggagatgttacaagattttgttagaagggtctttcccttctaaagtgtttggttcaagttatctaaatgtcaagagccgatattttgttattaagctcaattctttgccttgtttgggtgtttttagaagtaatcaagatgatctttaaatgtttagtttcacaaacattctaacctcggaattgggagtgctaatctgatatgaattcctttgacctggattgtcagtcaggaagatcatatggcaactggtatcgcttcagtaagcggacagttacatttgaggaagcctgtctactggaggagtagctatggaaaagctcagtgtcattccaatgtgatcctgaatggcatgcaaaaccagatcccttggtacgtattaggatgatgtttcttcacctatctctccttctctctctatctttccctgctgtattatcttctttctattgccccatctcctctcttctgggggaatgattgccaaaatattttattctggagcttttaagatgttattacatttcaaattgtacggagataggcattcacgcgttggctgttggactgtttattcctccaatgagaacgtactggaaagaatctttgtatacgtgtttaggcataaaccagtaatatctttttttcatgagataccagaatcctaaaagtttttcttttttagtcatttcctgattctttagaaaaaaaagaaaggttatcattttcattttctggtggtgatatgctacttaaattttccaggtcttattgggtttccaaattcttgcgagttcatagaagtaactattcacaatgtcaagtgaaaacaaactggaagtctcacagcggaacaatcaattcttgccagagagatggctcaactaggtatttcgatttcgcggtgattggtagtggaattgctggccttcgatatgctcttgaagttgccaaacatggaactgtagctgtgataaccaaagctgagccacatgagagtaacactaactatgctcaaggtggtgtaagtgctgtgctctgccctatggattcagtggagagccacatgcaagatacaattgttgcaggtgcttacctctgtgatgaggagactgttagagtaagttcacagaatgttattgtctcttcagttccatgaagcagtttgccctttttcagttttttctcattggagagtgtttccttttacttttccaaatttttcccggaatacttggttggatgaataggaaagttctccatctttcagtttgaaaccaaaggacctttctgtttagacggcttttgccacaggatctagagctgccaaaaattggaaaagagtaagagcaatggggcagttaggcttgttttcaatttgaagctgaagtgccaagcaacaatactacaagaaaggctctatgtctattccttgcttctgatataagtgcttaaaagttggaactgaagaaagagttggagagttgggaaaccaatggttggtaatatggacgatttccactggtttatgtagtactcctattctttatggttcagattgttgacttttgtctttgaacattagggaaagagagtgaaggtgacatgcaggaaagaagagataagaataagacaggaaattcacatgtgttgtatcttggtttgattttgggatttcatttagacagtaccatgttttcttcttttaaggagaacacacaaaagtacctttaacacttctgacttccctaaatcagcaccaattttttgagggtaactgctgataaggatagacactccaaggcgatccaggattcctagtcatataagattctctcctatccccacaagggtcctatgtgcagaaaactctatcccttctccctcgagctttaacctaggaatccatttgattatgtgaaaaagcacaagagaaaaatatattattgatttattaactatgttacaatgagccctatttataagtatacataatacatacaacaacaacaaccacccagtatagtcccactagtggggtctggggagggtagtgtgtacgtagaccttacacctaccctggggtagagaggctgtttccgataagaccctcggctctctccttccaagaactctccaccttgctcttggggtgactcgaactcacaaccttttggttggaagtggtgggtgctaaccactagagcaacccactcttgtcataatacataacctactcctattacatacgggactaggactaattatatatatatacacacataactatctaacactcctcctcaagctggtgcatataaattatatgtaccgaacttgttacatatgtaactaatacgaggaccagtgagaaacttggtgaaaatgtcagcaagttgatcattcgacttcaaaaactttatagcaatatctcatgcgagtattttttttctgacaaagtgacagtcaatctcaatgtgtttagttctctcatggaacactggatttgatgcaagatgaatagcagcttgattatcacacacaagtttcatctggcttatctcaccaaattttaactccttgagcaactgtttgatccaaattagctcacatattgccatagccattgctcgatattctgcttctgcactagaccgagcaaccacattctgtttcttgctcttccaagacaccaaattacctcctactaagacacaatatccagatatagaacgtctatcagaaggtgattttgcccaatcaacatctgagtatctaacgatctgctcatggcctcgatcctcaaacaataatcctttgtctcgggctgattttatataccgaaaaatgcggacaactgcatcccaatgactatcacacggagaatccataaactgactcacaacactcataggaaaggaaatatgaggtctaatcactgtgaggtaatttaaattaccgaccaaccgtctatatcttgcgggatcgctgaacggctccctcgtcctcgcagaagtttagaattcggatccatcggtgtgtcaataggtctacaacctgtcattcctgtcttctcaagaatgtctaaggcatacttccgttgtgagatcacaatatctgagctagactgagcgacctcaatacccaaaaaatactttaatctgcccagatccttaccctgaaagtgctcaaagagatgttgcttcaacttagtaataccatcctgatcattgccggtaataacaagatcgtcaacataatggaccagataaatacagagatttgaagcagaatgctgataaaacacggagtgatcagcttcactacgagccatgccaaactcctggataactgcgctgaacttaccaaactaggctcgatgagattgctttagaccataaactgaccggcgcaagcgacatacaaagccactagactccccctgagtaacaaactagatggttgctccatataaacttcatcctcaaggtcaccatgaagaaaaacattcttaatgtccaattgatagagaggccaatgacgaacaacatccatggataagaaaaggcggactaatgctattttagccacgggagagaaagtatcactgtaatcaagcctgaataattgagtatatcctttggcaactagacgggccttaagtttttcagcctggctatccggaccaactttgactgcatacacccaacgacaaccaacagtagattttcctgaatgaagaggaacaagctcccaagtactactcgtatgtaaagcaaacatctcgtcaaccatagcccgtcgccatcctagatgagatagtgcttcacttgtagacttagggatgaaaacaaaggacaaaaaagatacaaaagcataatgagggtgatgacgggcgatgataacttaaaccgacataatggggattaggattaagtgtggttcatatacctttccgaagtgcaatcggctgactaggaggagcaagtccgcagtaggagcagggtaaggtgcaggacgtgaatcagctgggcttgatgctgggcgcggacgacgacgataagtcaagagtggtgttcctgtggctggggttctaggaggagcaacactagattccttaacggtttgtgtgggtaagacttttgtgattgagaatgtaggaggagctatagttggtggggctagagctagaatggggctgtaggtgatggagacgtggaggaaggtgaaggggaaatagtgaatgaatctccaaaaagatggaactggtaatacctcaaaaatgtctaagtgaccacctaggcatgtgaagtatgactgagtttcaaagaaggtaacatcagcagacataaggcactgctggaggtcaggcgagtagcatcgataccccttacctaaaaatacacacttaagagcacggggagctaacttatcttttcttggagtaaggttatgaacaaaacatgtgctcccaaagacacgaggtggaagagagaagaagggtgagtgaggaaacaacaaagagaatggaacttgattctggatagctgagtatgtcatacaattaataagataacaagatgtgagaactgcatcccccaaaaatcgcaacggaacatgatattgtatgagtagggtacgggcagtctcaatgagatggctatttttcttttccgctaccccattttgttgagatgtatatggacaagatgtttgatgaatgatcttatgagatttcataaactgctgaaatataggagacaaataatctggggcattttcactatgaaatgtgcggatagaaatcccgaattgattttgaatttcagcacggaaaacaactcagatcgatttttcatcaagaatatccaagtgcacctggaataatcatcaatgaaactatcaaagtagcggaatcccaaggtagaactgacctgactaggatccctaacatctgaatggactaaagtgaaaggtgactctgctcgattatcagagcgtcaagggaaacgagagtgagtatgcttaccgagctgacatggctcacacactagagtgtacaagtgagacaaatcaggtaccattttctgaagttttgataaactgtgatgtcccaactgtttatgtaataaatctggtgaatcagtaataaaacaagttgttgatatgggttcatgtgatttagcaaggataaggtaataaagtccatgtgattcatgtccggtaccaataatccgccccgtactgcattcctgcataaaaacaaggtcatcaagaaataaaacagaacatttaagtgatttggctaagcgactaacaactatgagattaaaaggactaccaggaacataaagaactgaattcaaaggtaaagaaggaagtggacttgcttgacctattccagttgccgcagtttgagacccattggccattgtgaccattggaagagattgatgataagaaatagtagtgaaagcagatttattaccatatgatgagacgctcctaaatcaataacccaattactgggagaagaagattgtgagacacaagtaacgctagtacctgtttgaacaacattagcaatctcataagatgtcttttacatgctttgtacagaaggaactctatatattccgataaagaaaccatctggattggattcaatgcattggatccgacggatacaaatgacattataatgttcacgctggaaaaatcagaaaatattctggaaactactgttcacgccagaaaaatatgaaagtggtaggaatttggtttaaattggatgggtaggctcggaattgcaaggtaaacaagttgtcctgaagagtcgtcgccaaaaaagggccgaaaatagccccacgcgcgtcgcgtgacatctgaacttagccggtaatttttttttctgtcggcgtgtgagggcgcgtggagggtggtctgtcggagatatttttacgggttggtcgtcaaaggctgatctacttcgtggtggtgttggtttttgcacaacactgatgaaaagtggttagttcttgcggtagacctgtgtttgctggaaagacttccggttgactgatttctcttcccggccgctggaatttatgcacaacgataaatctctcacgatttctctaatagcatgtgagaaagcacgggagaaaaatatattattgatttattaactacttataagtatacataatacataacctactcatattacatacgggactaggactgattatatatattcacattctaacaaattttcttaatgctaacaactcatgcagagttgtgacatgcccaattctgctgagagtagtaaggcccagcggatttcgcatctactaggcccattaacaacatacaagagggagaggggatagagttctctgtacataggactcttgtggggataggagagaatcttattatatgatacaacttaagctaggaatcctggatagcctgggagtgctgtatattattttcatttgtctctgtaaatatatactggcttcaaggaagttttgcgttcttgggtgacgggacatcacaactggtatcttcttatcagttgagataatcgtcgtccatgcaattgtactttttatgcagtctctgtgctaaatgaatttacaagatgactgatttattactccaacattgtgtttagtatactcttttgaagtcttcatttttataagtgtatctcctttctccaggttgtgtgtaccgaaggacctgagagaattaaagaactgattgctatgggtgcttcattcgatcatggggaggatggaaatctgcatctagccagggaagggggccactcccatcgtcgaattgtccatgctgctgatatgactggcagagagatagaaagggccctattagaggcagtttttaagcatcctaatatacatgtgtttcaacaccattttgctatagatttgttgaccactcaggtaagtttattagtgtgaaaattttgctatagttgtgtaaaggtggcaattgaactgttcagtaaggatttaatgttaatttgtatgccaaatgcaggatggttctgacatagtatgtcatggcgttgatactataaacacggaaacacaggaggtaagtacagttgctttcactcatgttaacctccatgttttgaacatttcctcaaaatgacataaattgatttctttggcttctgcgctcttattttgagtttgcaggttataagattcatttcaaaagtgactttgctggcatcaggtggagctgggcatacctatcctagtactactaatccgccggtatgggtttcaatatcttttccttcataatgttgttagttatgagggcactccttgtaatcagtaagattattcagtcctaaacagtgatatggggggagaaggtggggaagggaatccctggtgctgggtggctaatagttacttttatgactagcatacatatgcatttagttgttggcgataagcttcgtcacaaagtatcattcgtaattcataaggaccttaacaattgacattggtgcaaacaacattccatagagtatgaaacatggcctgatttaaaaccctttcatgttaagctaacgtgctaattagaaataacagctgactgccctaagtcacaaaaaagggacaagtccaaatttacccttgtactttgcgaaaaggtttagatttatcatccggttgaagttagtttggctcactagtgcctcgctgttaaacttttggacgatatttacccttatttgctaaaggacctttgtttgaggtttaattgtctctaagtatactgaataacaccagagactgccacgtgtcccacacgtggcctgaaattaatccctcccctttaacctgaccccgtttgaccctgaaaagtaacccccctctcactaaaattaaccacccctcttacccccacccttttaccacaaacaaggtggccaacggaaaaacaactcctacactgtccgtcttcattacacttctgcaaccaccaaacaacctcaccaacccaccaatagcaccccagagactcactgctcctccacttcaaccctttctcggcgaacaccttcccctcagttccacggatctcaccaaaatagaaccttcatcagtcaccaccattacaactgtttacccgaaaaacggatagagttgaatttattcgtagttctaaggatatgtgatatagctcaatacaaattgtaaggataaaaggaaaatatcaaatatggaccgcaaagaagactaaataaacaaagttgtaacaaaagcgatttttgggaccaagcaagatgaatcagtttatgaggcttaaaagaataactctcgaatatcagagaatatgttgcttgaattacaatctaaactccaaaaaaactgcccttccagaaatgataaaacccctctttatagtagagggaccttactttaaatataattaaaaaatactcagtgggagatccatgataaatcaacttttccacaattcctgccaagattctctcatctagtgggattgcaacggcttatgtctgtgagtccgatctgactcgggcttttgatctcggcttgagcttgattctaactcgagctctcgatctttggcttaagctcgattctaactcggacccttgaattgattcggggtcaatgttggttggtctctagctcataagcttgatagctttactctgcatcatagttagatttggatttgagctcaataacaatatcgaactcgacattgatcggcccctcgggttcgaggcttgtttgttccatcttcggaaactatctcgaagtctcacttcgatcgatcatcattcgaactcgatcagacgtgcgaaggccgaaatctatttcgaccgtatacagatagtcccctcgcttcttagaaagaatgtggtgagaaacgatatgatcttttaacggctcgatcggattataacctgacgtttccatcgggctcgatcatgacgcatatgatagctgttccgtcggtttagtctttcaaggcatttaatgcatgtcagatggtggtcggccactgctgatactgaaccgccatcgcttaaacctataaataacccttccttttatcatttaccacttttacatcttcaatcttccaaatttcccaagtcccttttcgcattacccgtaaatctgtgatttctttttacaaaagcccctcttcaattctaccaaatctttgtcactttcttctattcctcacttttgaattcgaaaatggcgaaaacatcacaaaccattcctcagaaagagaaggcttcatcttcacaatgtgctgccgataagacaccagcaaaaccacgatctgaggagtgcgttctcggggcgtgtgttcttacttctgattttaaggtcgataaaggctcatcggtccctggccgatgtgagccagtatcgaggtacatatgttcgataaccgagaagcacctcaaacagctaaagaaagattgcaattgggataaaaaagaaataatgattccttcttctgacgaagatatcacttcttacgtgaaagggtttttgaatgtgtatacttaccctttcacgttaggtcccctcgattccgttattattgacttctgtcgtcaataccaaataaccataggctaggtccatccttctttctggcggatcgttatcctgatccgatactttgtgagcaaaatcgaggggatgccgttcaccctcgaccatcttatccgattgtaccgtcctcgactttttcaaggagggttaataaaacttcagcgtcgggctaccaaggctctgttctcgagcattgacgaggacagggatcggggctggatgggcaggttcgttcgagtgaggacttcggacctgattccgaccgaaaagatgccctttcccgaggagtggaatatgaaacgtaagtgtgatcctgctgttacttctattttgttctttcatttcttttctcaacgacactcttctttttgtgatgtagcggttccctggatgcccggagcagttctcgatctcaagaactgggtacgagctcttgtttcgacctttacatacgccgagcgctcatgccgtgatttgtcaaagggtggtgggaggccaagaatcatggtaagcccctttctagtactctttgataattcgaacgaggtggtttccaaatattttaataaattttttcatatccaggtttgggcaaagatgcagttttgaggcccttgtccaacgaggaagaaacttcggcctctgttccaaagccggtgaagggaaataaaaagaaaagagccaccgttcccgaagatccaaacccgaagaagaggacggctcgtaagccgaacaagaatgccattcctttgaccgtggaatcagttctgcgtctaagggatgaagatgaagaagaagaagaagaagaaaatgatgggtccgcgctggcggcccgaacgaagagaaccaccgatgccccatcggcagctggatcgatgatgctttatgaggctccgcctcgaactgaggatataccggagaaagattcgggtggaatccctgaattatcggagatcgaagacgcatctcatcggagccaacgggtgggtgatatgtctgaaagggccctcgaatcccttcgaaccgaagagaatgctccaagtaattcattttggggcagcagcaatcgaagattcgcccacctttcccgcttttttcgcaggggtgattcgggaagcccaagctctgggggccctcgatctagataggcctcacgatgaagaggatccctttcgtgacctgtttaccggtatcgaggacgttgccggcactggtgatgaatcagatctttttcacggggtacggcaggctttgaatcaggtaagccttaaaattattttgtcggtactatctttatgtttacttttcattaacttcgtttcttgtttctttgtaggcaacgacagtttatcgagaagcatgttctcggtcccaaaaagcgctgcgtcgatacgaggccgaccttcaacgggttactgatgagagaaactccctaacacttcttttagggcagagagaagaggaaataaaagacctccgagctgagttggccaaggcttatcgagatcaggccgatttgtctgagcaggtaatgatacttttaaaagcctatgggcttgataccggaacgatggctaatttttcggtctcacagttgcagcaaaaaattgagatgatcgggaagcttcgtgaggaggtcgacgtgataaaaacagagtctttgcagtggaaagaaggtatgaaccgctttgatgcagagaaagaaactgctcgagcctagttatcatctgccgaaacccaacttcagagaatgaaagaaaaaggcctggttcaagcaagaagaatagaggagctcgaggctcggttggcctctgtacttgccaaggccgaatctgatgccgaaaaggcaaaagccgatgcggatgcactcgtggccgtctatcgggccgatgctgaagctgcccaggtctaagcaagagaggcagccgagactgccgatactcgagcacattgggtcgccgaacttgctaagtgccgatctcggagggaaaccctcgaggagatccatgctcgtggtttcgatctcgctgaagagataaaaagggccaaagaactcgaagccgatgctgaagccctggtttccgatgacgatgatgatgatgacaatgatgatgatgatgggagtaagagcggatccgagaacgggggggagcccgatagagaagagaccgctcctgaggatgaccaggaagcttagtccttaatttttacgttgtaatcaatcatgtagacaattttgtatatagacaatattgccgacttgcttctgttttgtgaagactttattcatgccttatgaatgttttcacaaggatttcaacaacttaatcaaatttggacttcgtagcctctataatcgagcgagtgcttattcaaacttgaagtgatgtagcccttaggcttattagttgagtcaatgattcgagctcgaagaaatatagcccgtaggcgtaatggtcgagtgggtgcttgctcgaactcgaaataaaagtagcctgtaggcttagtagtcgagtgaatgattcgaactcgaagtaatctcgaagtaatgtagcccataggcgtaatggtcgagtgcgtgcttgctcgaactcgaaataaaagtagcccgtaggcttagtagtcgagtgaatgattcgaactcgaagtaatgtagcctgtaggcgtaatggtcgagtgcttgcttgctcgaactcaaaataagagtagcccgtaagcttagtagtcgagtgaatgattcgaactcgaaataatgtagcccgtaggcgtaatggtcgagtgagtgcttgctcgaactcgaaataaaagtagcccgtaggcttagtagnnnnnnnnnnnnnnnnnnnnnnnnnnnnnnnnnnnnnnnnnnnnnnnnnnnnnnnnnnnnnnnnnnnnnnnnnnnnnnnnnnnnnnnnnnnnnnnnnnnnnnnnnnnnnnnnnnnnnnnnnnnnnnnnnnnnnnnnnnnnnnnnnnnnnnnnnnnnnnnnnnnnnnnnnngtaggcttagtcttgaactcgaaataaaagtagcccgtaggcttagtagtcgagtgaatgattcgaactcgaagtaatgtagcccgtaggcgtaatggtcgagtgagtgcttctcgaactcgaaataaaagtagcccgtaggcttagtagtcgagtgaatgattcgaagtcgaagtattgtagcccgtatgcgtaatggtcgagtgagtgcttgctcgaactcgaaataaaagtagcccgtaggcttagtggtcgagtttatcttaattctgtttgcataataaatctccaaatagaggaatttttcttggatataagatgttggcaaagaggagaactttctttgcaagtcactatacatgtgtttatgtttcgtgtctgggttcgggccaactacatgagcatggatcgttttgaccatttggcttttacaacttttcctattggaaacccgttgttgcgaaataactttcttgcatcagaatttgatatattcgagggctaatgccccccagtattcgaggtcgattgtaaagaggcctcggatactgttgtaagcgcagcacgatcattggttgcctcattaaaaaccttgccgaaaaacccatttgggataaaaccggtctaagggaaaaagagtgcaacacgtgctttcagatcttaaggcttcgtattgaaggatccatcttagctcctgatcgaacttctgcaggggtcagttttagaatgtaaatgaatatgggagggtcgtaccttagcagtagtatcgttttagatgtgacacattccaattgcttgataattgtttgctgtttataatgccgagcttgtatgatccctttccgacgttctcgagaacctgatatggtccttcccagttcggtcctagttttccttgttcggatttcgggtattgagggtgactttccttagcactaagtcctcgggcttgaaatggcggagcttggttcttcgattataatatctttcgattcgttgcttttgggcggccaattggacgagagcagcttctcgttttttgtccaataattcgaggctagtgttcatagcctcgttatttgattcttctgtcgtgtatcgaaatctggtactgggttcgccgacttcgactggtatcaatgcttcggacccatatactaaggagaacggggttgcccccgtactggattttgacgtcgttcgatatgccctaaggactttgggtaggatttctctccactttcttttagcgtcgttcagcctcttctttaggttttgaatgatagttttgttcgttgattcgacctgtccgttcccactggggtgatacggtgttgataatatccttcttattttgtgatcttcgaagaatttcgtcactttgctgcccacaaattgtttcccattgtcacatactatttcggcgggtatcccgaatcggcatacgatatgatcccagattaagtctataacttctctctctcttactttctcgaacgcctgtgcttcaacccatttagagaaatagtcagtcataaataaaatgaatttagctttacctggggtcgatggcagagggccgacgatatccattccccatttcatgaatggccatggggataggaccgagtgaagttgttctccgggttgatgtatcattggcgcaaacctttgacatttgtcacattttcgaacaaatgccttcgcatctttgcccatatcgatccaataataccctgccctgattattttttcggactaatggatcgacaccggagtgattcccacaagtgccctcgtgcacctcacgtaagatgtaatcggtatctcctggacccaagcatactgccaatggtccatcgaatgtccttcggtatagcgttccatctgaagccaacgtgaatcgagcagctttagtccgtagggcccttgaatctttaggatccgatgggagctttccgttctttaagtattcaatatacttatttctccaatcccaggttaagctcgtagaatttatctgggcgtgtcctttttcgatcacggatctcgagagttgaacgacagtccccgagctcaaatcaccttcctcgaccgatgatcccaaattcgcaagtgcatcatcctcactgttttgctctcgtggaacatgttgtaaagtccattgtttgaaatggtgcaaagtgacatgtagtttgtccaaatacctttgcattctatcttctcgaacttcgaaggttttgtttacttgacttaccaccaacaagagtcacatttggcttcaatgacttctgctcccaagtttttaactagctcgagacctgcaatcatgacctcatactcggcctcgttgttagtcaacctggtagttttaatagattgcctaatagtgttacccgtgggtggctttaaaactatgcctagcccggaccccttcacgttcgaagccctatccgtaaaaagggtccataccctcgatgacgtacccgatttcaacaggagttctttttcgacttcgggtacgagggttggcgtgaaatcggccacgaagtctgctaaaatttgagacttgatggccgtatggggttgatattcgatatcgtacccactgagttcgacgatccatttggccaatcggcctgatagttcgggcttgtgcaaaatattacgaagtgggtaagtcattaatacgcatatggggtaacattgaaagtacggtcgtaactttctagaggcgcttatcagtgcaagtgccaatttttctaggtgcggatatctagtttctgcttctcctaaggttcgacttatataataaatgggaaattgcgtaccttgctcttcccgaactaggacaccgcttactgcgatttccgatactgccaagtataagcaaagtttttcgtctgtttttggtgtgtgaagtagtggtgggctcgacagatattgttttagttcctttaatgcctgttggcattccggggtccaagcgaaatcgttcttctttttgagtagggagaaaaatttgtgacttcgatctgatgatctcgaaatgaatcggcctaaggccgcaatccgtcccgttagcctttgtacaactttcacgctgtccacgatggtgatgtcttcgatggctttgattttatcagggttaatctcgattccccgatttgacaccatgaagccgaggaacttgcccgaaccgaccccggaagcacatttttcggggttgagcttcatgttgtatttcctcaaaatctcgaacgtttcctgcaaatgggtcctctgcgcgcagggatttaactagcatgtcatcaatataaacttccattgatttacctatttgttattcgaacattttatttactaagcattggtaagtagcccctgcattttttagcccgaagagcatcacattataacaatatgttccatatttggtgacaaacgaagtcttttcctggtcctccgagttcatctggatttgattatacccggagtaggtatcgagaaaagtgaggatctcgtgaccggccgtggcatcgatcatgcgatcgatgttgagtagcggaaaagaatctttggggcatgctttgttcaaatccttatagtccacacacattctaagtttattcccttttttaggcactacaactatattggctaaccatttgggatatttcacctcccgaatggaccctatcttgagaagtttggttacctcgtcttttatgaatgcgtgttttacctcggactgaggtcttctcttttgcttcaccggtctgaacttagggtccaagcttagccgatgcgtcgttatgtccggtgggatccctgttatatctaaatgggaccaggcaaagcaatcaatgttatcgataagaaattgaataagtttcttcctgagttcggggctcaaccccgttcccaggtatacctttcgttcgggccagtgctagattagtgtgacttgctccggctcctcaattgttgatttggtggcgtcggatcgagggatcctctgatcatcatcttcttcgatcttccggttatctggctgggtcgaagccgatgtctgtgattgctatttggtatctcgttctccttctgagcccgatccctttattggtgaaggcgaggatattggtttcgcttcctcgacagcgaacatttcttttgcggctggttgttctccgtacactgttttgactcctctcgatgttgggaatttgaggacctggtgtagggtcgaaggtacaactctcatgttgtggatccatggccttccgaaaagggcgttgtatctcatgtcgccttcgatcacgtgaaacttcgtttcctggatggttccggccacgtttattggtagaattatctcgcctttggtggtttcacatgccatattgaatccgtttagaaccagagttgcgggtacgatctggtcctgcaggccgagctcttctacgaccttcaatctgatgatgttggccgagctacctggatcaatcaacacacgcttaactttagttttattcatgagtacggatattaccggtgcatcgttatgaggttgtatgactccttctgcatcttcgtcattgaaggacaaagttcctatgggtgtgtaatcttgagttcgagatcgattttctctcacaatcgatgttttagtgcgtttaagcactagtccctgaggggtatcggcgccgccaatgatcatgtgaatgacgtgctgtggttcttcctgttcgttttgcttgccgaaatccctgtttttaaaatggttcttcgccctatcgctcaaaaattcccgaaggtgccctttgttgaataaccgaactacttcctctcttagttgcctggaatcttctgttctgtggccatgggtgccatggtattcgcatatttgattgggattcctccgggcaggatcggtttgcatgggtcgaggccatttagtgtctttgatgcgtccgatagctgatacgatggcgtatgcatcaacgttgaagttatattccgataaccgaggtgcttccttagatccgacaggcctatcgaaactacttctgtttatcagcccccgggacccttgacctcgatcactttttttttattttgcttgaggttatgtctcgattcaccgactctgtggcttccgttgtacggttggtatcgatccccaatcagacctcgttctcgattagtatcccttcaattagcgggttcagaccccaattgatcatcttcgaccctaattttcgattggtaccgattgtgcacgtcggcacatgtgatggctgggtattcgatcaggttatgctttaattgccgtgaagccgtcgaacttcgctcgttcaaaccttgagtgaaagcctgaacagtccaatcgtctgtgactggtggcaagttcattcgttccatttgaaaacgagatacgaactctctcagcatctcgttatccttttgtcttaatcttgaagaggtccgatttccttgttgcgacttttatggcgccgacatgtgttttcacaaaagaatctgctaacatggcgaacgagtcgatgaaatttggcggtaggttgtaataccaaatcattgcccccttcgagagggtttctccgaatgtttttagcaacacagattcgatttcatcgtcttctaaatcattgcccttgatggcatatgtgtaagaagtgatgtgctcgttgggatcggtcgtcctgttatatttgggaatttcgggcatacagaattttttggggattgctttcagggctgcgctcgaggaaaaaggtttttgcacgaattttttcgaatacaacccttttatcattggtggagctcccgggatctgatcgaccctagagttataagtttctacttttttatcgttggtttcgactcgctttgtgagttcctcgagcaatttagcaatttcgggagtagtccccgattcttgctcatttgactttactatggctggttccgttctgtgagtgatttctcggggtggattgggctccggcctgctttgtagctgggtttggctctgcaactgagctattgctgcctgttgggcttgcaacatttcgaaaatcatacgcaagttaacgccgttttcctcgatgttttgggtatctcgagccgcagaccgagtgccaccatggatgctattctcgggttcagcatgtaggttcgcctcaatggctacatgcgaattgatatcaattggcgctccgattcgagctccaacggtgttcacaagtggtctttcagtactgggtgtcaagttgttttcgtcttgaagaccggccccgttatcgatcggtgaagccatttgattgatggttagtcgtagctaatccgaaattcaagatattttcggaaacaagcgtaaaacacaatggcgtgttttttcagattcgtatcaaataaccactgttatccttagccccacagtgggcgccaaactgtttactcgaaaaacggatagagttgaatttattcgtagttctaaggatatgtgatataactcaatacaaattgtaaggataaaaggaaaatatcaaatatggaccgcagagaagactaaataaacaaagttgtaacaaaagcgatttttgggaccaagcaagatgaatcagtttatgaggcttaaaagaataactctcgaatatcagaaaatatggtgcttgaattacaatctaaactccaaaaaaactgcccttccagaaatgataaacccctctttatagtagagggaccttactttaaatataattaaaaaatactcagtgggagatccatgataaatcagcttttccacaatttctgccaagattctctcatctagtgagattgcaacggcttatgtctgtgagtccgatctgactcgggcttttgatcttggcttgagcccgattctaactcgagctctcgatctttggcttaagctcgattctgactcggacccttgaattgattcggggtcaatgttggttggtctctggctcataagcttgatagctttactctgcatcatagttcgatttggattcgaactcaataacaatatcgaactcgacattgatcggcccctcgggttcgaagcttgtttgttccatcttcggaaaccatctcgaagtctcactttgatcgattatcattcgaactcgatcacacgtgcgaaagccggaatccatttcgaccgtatacaacagctttacaaccccatcaacgagccgcccctctaccatagcaaaacccatcgtctttcatttttaatggttgatggtgtcgcatagggaaatttttccggcgacatttttttttattttttaaatttttgaaggttctgtggtctcaaacttttatgaaaatttcagggatggttaattatggttggggtggttgctacctagagataacggtggaagtgattgtttaggtatagagggagtactttgggtgacggtggagaatggtttggggtgggattttgggaagctattgcttgagtattggatggtgaaagttaactagatgaagtgggtttggggcagcaacatgttgggcaatagaagcattactgtgttgcaatggagaaggggaatagatggagctcttcgctggaagttgggcaaaatggtctaagagcagtgccggggtgcaggggttaaagggagagggttaaaggggcagggaggtttattaattagccacttgtgggacatgtgacacattttggtgctaaacagagtaattagatattaattaaaaaaagagattaatcaactgttagcaaataagggtagatatagtccaaaagtttaacggtgagggcatcagtgagccaaacttcaaaccgagggtaaatctagacctttttgcaaagtacaaggggaaatatggaacacccccacccccccacccccaaannnnnnnnnnnnnnnnnnnnnnnnnnnnnnnnnnnnnnnnnnnnnnnnnnnnnnnnnnnnnnnnnnnnnnnnnnnnnnnnnnnnnnnnnnnnnnnnnnnnnnnnnnnnnnnnnnnnnnnnnnnnnnnnnnnnnnnnnnnnnnnnnnnnnnnnnnnnnnnnnnnnnnnnnnnnnnnnnnnnnnnnnnnnnnnaaaaaaaaaaaaaaaaaaaaaaacttaaagttctgggtataatagatgatcctttccttggatgagtggattcttgtcaagacacattgttcaacgttgtaataacctgggttaggcatctgctgtggcgttgttatgctcgttatcaaatttgcctttcttttgaaatcatttctgtaagtttttggagcaactaattggcggtggggccaattctgtttttatatttgacaacttgtgcctttattaatgaaaaaaaaagtttttttaatgtgggcatgatggttgtaggttgcaactggagatggaatggctatggctcatcgagctcaagctgtaatttctaacatggagtaagtgatcctcagttgcattgcattctcattgtacaatatctctgcccctgctttagtgagttgtgctgtaaaatctgctaatcttgatttcatcctttttttgccttcttgatttctgcatcttgttctgctattcattcagaatttgcacttttgactaaaaatacaagggtgtgttcaaaatgttgtgcgggatgatattggatatgcaacttgaatttttcaggattaagggcatcaaattttcttcattgagggatttagttgatgtagaaaagatttctagactagcagtctgctctctaattgatggtcctcctttgatcatcttttggatggtagacaagtctttatttgcgaggttgatgaaggttgcattagtaattacaattctcttcctcgtgttgccaggtttgtgcaattccacccaaccgctttggctgatgaaggccttcccatcagaccaacaagaaccagagagaacgcttttttgataactgaagctgtcagaggtgatggaggcatcctttacaacttagatatggagagatttatgccaatgtatgatgaaagagcagagcttgccccgagagatgtggtagcaagaagtatagatgaccagctcaaaaagcgtggtgaaaagtatgttcttcttgatatcagttacaagccccgagagaaggttctttctcattttcctaatatagctgctgagtgtctccgccatgggttagacataacacagcagccgattccagtggttcctgctgctcactacatgtgtggtggagtccgtgctggactcgagggtgagactaacgtgcatggtctttatgtggcaggtgaagttgcatgtactggtttacatggtgcgaaccgacttgctagcaactcgttgcttgaagcactagtgtttgcacgaagagctgtacagccttcaattgatcacatgaatgtgtctagaattgatcacggtgcttcaagttggtggtcgcggcctgtagctcccatgttactaggagatacagtacatggcaaagtcattcaccggacaagggaagtaaggaaagaactgcagtcaatcatgtgggaatatgttggaattgttaggtctacctcaagactaaccgcagctgagaagagaatcagagagttggagttggaatgggaaacatacctatttcagcatggctgggaaccaacaatggttggagtagaggcttgtgagatgaggaatctcttctgttgtgccaacctggtagttaacagtgctctttctcgacacgagagtcgcggtcttcattacaccattgattttcctcatgttgaggaaagcaaaaggttgccaacgatcatttttccgtcacagcgaaatagctcatggagctcgcggcaattacacaggcagcagatatgttagatgctcttacctatttgccaatccttcctgctaaaacttgtcaagcgcagtgcatgattagtttttaggtaaagaagatgctcatgggttattgtcattcttcccgccattacatttggggcagggcaatgtcattctttggtgaaatatatatatatatatatatatatatatatatatatactgtagacaataaatttgcgtcaggaaaataaaatcaagctgaaaaatattgcaacaatcgtagtattttatttcaaatatttgagtgttacaatctgtatgaatcctctgattcttcttttcaacggtaaataaaagagcctttgagcttaatcttgaattttaatttattttaatccatgtgtttggggcctaatcttgatcttgacgtatttttaatccaagggcttgcagcttgttcttgaatcttcgtcttgatcttttaatccgtagaacacttgaatgcttgtagcttttagagaaatctgcagcgtttgatccacgagctccctcttgctttttgttataacttctggtcccctttctgggttgtgaaaaccctcatttatagttgtggaagggagaagttgtgataagaacaagctctttccgaccaatcagattgaggagtgacaatgccgcatttgattggccagaacatgtcacttgcatatgtggcgcgatttcattggccttttaatgtgacttggcatgacttgtcattttgacacgtggcatgatcatattggctctttcgtttgacttggcgtgccacgtcatttgacatgtggcaccaaactgggcctctaggaagatgacatcttgggctcatcactttagcccaattaaatgggttagcccaatggattaagacttatttatttaatccataaaaatgggacatatacaattaatccacttatattagtccaataaatttatttgaactaatataacttgaatttcaaatatagtacaaattattttatgaatttaattttaataaaatttatatgtctacaaatgctccctacttcaagacttgtcagaacatagaagactaggcttgaaataccatgaatgcatgcaacggtcattaataccccataactccaatatgaaggaaatttcatgtcttatttcctttaacgtttctgggcattaggacgagctttcaaagttttaattctccaaatccaaagatttgcccagtacagatttgattaaggaatctttggatggttaattgctttcttcttttttgtaatttcaaacaaagtgccaagaaattttgagatgataaagtgcacggaattaagatgggatttatattgacttgagctttcctagccatgatgcagcatcttccataagaaacttttgcaagaattatagataacatctccaacttcacgtggcttaacaaggaaactacatactgctaatatagacttccacactcttggcaccaattagaacaccgccactactagtagccgaatccttgttggataaaaagttagtctcgccgctttgcaacttattcccacatcggcagcatcattgtaacatcttctttcaaagatctatataaacccgcgtgctcgtatttgttcaacatccattcgcagtatttgcaagccacttgagtctacctttgtgaattcggaagcattaacgctgaggtaatatcttcttctttttttgtgcctttttttttcactccgttgtctcttttttaaaagtaacttcgtcaaactacgaagccctttataagttcaagatgaaggcctttaaaagtccgtgatgaagatctttaaaatttgcggcggcaaaccataaaagttcgtgatgaagacctttaaaatttgtggcgaaaatccttaaaagttcatggccaagatttttaaaagttcgtggtgatgacttttaaaaatttgcggtggagacctttaaaagtacgcgatgaagacctttaaaaatttgtggcgaagacctttaaaagttcgcgatgaagaccttaaaaatttgcggtgaagacctttaaaatttgcagcggaaaaccataaaagttcgcgatgaagacctttaaaatttgcggtggaaaaccataaaagttcgcgatgaaaacctttaaaatttgtggcgaagatccttaaaagttcgcataaagatccttaaaagctcgtggtcaagatctctaaaagtgcacagtgaagacctttaaaagttcacggtgacgacctttaaaagcatgcgatgaagacccttaaaagctcgcgcaaagatccttataagttagtggtcaagatatttaaaagtgcacattgaaaacctttaaaattcgtggcgaagatccataaaagttcgtggtagaaatctttaaaagtcggcagtggggactctttaaagttcgccacaagcaccttcaaaagttcaagacaagcacctttaaaagttcgaaacatacgccttttaaaagttcagaacgaaaaccttaaaaacccgaatgccattaaaagttcgagacgaacacctttaaaagttcgcaacgaaaatctttaaaatttcgaatgcctttaaaaaattcgagacgaacacctttaaaagttcgcaacgaaaacctttaaaacttcaaatgcctttaagttcgagacgaacaactttaaaagtccgcaacgaaaaacttaaaaaaagcaccttcataattgtccctgactacattttaaaaccaactttatattgcaccacgctgccaatttcagatttgcgcagtctcatcaaaatattcgtatcttggtgtagaaatatcgaaattacaaaccatttgatttcttggaaactagacttcaaaatctaaaacatgtccaaaacgtgcgatttaataccttaaggatagtttcagataatattttgaagtcaacttaaaatttcgacacggtgacaatttcaaacttgcgcgattttaccaaaatttttatatcttgatgtaagaat